European Patent Specification EP 3 490 583 B1, published November 29, 2023. Title: ONCOLYTIC HERPES SIMPLEX VIRUS VECTORS EXPRESSING IMMUNE. Applicant: Virogin Biotech Canada Ltd. The sequence listing filed with the application follows.

SEQUENCE LISTING (575 sequences)

SEQ ID NO: 1 - protein, 335 aa, Mus musculus
MCPQKLTISWFAIVLLVSPLMAMWELEKDVYVVEVDWTPDAPGETVNLTCDTPEEDDITWTSDQRHGVIGSGKTLTITVKEFLDAGQYTCHKGGETLSHSHLLLHKKENGIWSTEILKNFKNKTFLKCEAPNYSGRFTCSWLVQRNMDLKFNIKSSSSSPDSRAVTCGMASLSAEKVTLDQRDYEKYSVSCQEDVTCPTAEETLPIELALEARQQNKYENYSTSFFIRDIIKPDPPKNLQMKPLKNSQVEVSWEYPDSWSTPHSYFSLKFFVRIQRKKEKMKETEEGCNQKGAFLVEKTSTEVQCKGGNVCVQAQDRYYNSSCSKWACVPCRVRS

SEQ ID NO: 2 - protein, 162 aa, Homo sapiens
MRISKPHLRSISIQCYLCLLLNSHFLTEAGIHVFILGCFSAGLPKTEANWVNVISDLKKIEDLIQSMHIDATLYTESDVHPSCKVTAMKCFLLELQVISLESGDASIHDTVENLIILANNSLSSNGNVTESGCKECEELEEKNIKEFLQSFVHIVQMFINTS

SEQ ID NO: 3 - protein, 267 aa, Homo sapiens
MAPRRARGCRTLGLPALLLLLLLRPPATRGITCPPPMSVEHADIWVKSYSLYSRERYICNSGFKRKAGTSSLTECVLNKATNVAHWTTPSLKCIRDPALVHQRPAPPSTVTTAGVTPQPESLSPSGKEPAASSPSSNNTAATTAAIVPGSQLMPSKSPSTGTTEISSHESSHGTPSQTTAKNWELTASASHQPPGVYPQGHSDTTVAISTSTVLLCGLSAVSLLACYLKSRQTPPLASVEMEAMEALPVTWGTSSRDEDLENCSHHL

SEQ ID NO: 4 - protein, 234 aa, Homo sapiens
MAPRRARGCRTLGLPALLLLLLLRPPATRGITCPPPMSVEHADIWVKSYSLYSRERYICNSGFKRKAGTSSLTECVLNKATNVAHWTTPSLKCIKPAASSPSSNNTAATTAAIVPGSQLMPSKSPSTGTTEISSHESSHGTPSQTTAKNWELTASASHQPPGVYPQGHSDTTVAISTSTVLLCGLSAVSLLACYLKSRQTPPLASVEMEAMEALPVTWGTSSRDEDLENCSHHL

SEQ ID NO: 5 - protein, 231 aa, Homo sapiens
MSVEHADIWVKSYSLYSRERYICNSGFKRKAGTSSLTECVLNKATNVAHWTTPSLKCIRDPALVHQRPAPPSTVTTAGVTPQPESLSPSGKEPAASSPSSNNTAATTAAIVPGSQLMPSKSPSTGTTEISSHESSHGTPSQTTAKNWELTASASHQPPGVYPQGHSDTTVAISTSTVLLCGLSAVSLLACYLKSRQTPPLASVEMEAMEALPVTWGTSSRDEDLENCSHHL

SEQ ID NO: 6 - protein, 353 aa, Homo sapiens
MRLAGRQVPEQRSPPPPGLGSARPGSPAVSCGAAAMAPRRARGCRTLGLPALLLLLLLRPPATRDARDRLAVLAGRSRISESFNHEVQTHEACVRLRTMENCPQCHHHRTSRQQAGITCPPPMSVEHADIWVKSYSLYSRERYICNSGFKRKAGTSSLTECVLNKATNVAHWTTPSLKCIRDPALVHQRPAPPSTVTTAGVTPQPESLSPSGKEPAASSPSSNNTAATTAAIVPGSQLMPSKSPSTGTTEISSHESSHGTPSQTTAKNWELTASASHQPPGVYPQGHSDTTVAISTSTVLLCGLSAVSLLACYLKSRQTPPLASVEMEAMEALPVTWGTSSRDEDLENCSHHL

SEQ ID NO: 7 - protein, 7 aa, Artificial Sequence
  Synthetic sequence
  misc_feature: Synthetic sequence
KVSALKE

SEQ ID NO: 8 - protein, 7 aa, Artificial Sequence
  Synthetic sequence
EVSALEK

SEQ ID NO: 9 - protein, 35 aa, Artificial Sequence
  Synthetic sequence
KVSALKEKVSALKEKVSALKEKVSALKEKVSALKE

SEQ ID NO: 10 - protein, 35 aa, Artificial Sequence
  Synthetic sequence
EVSALEKEVSALEKEVSALEKEVSALEKEVSALEK

SEQ ID NO: 11 - protein, 96 aa, Homo sapiens
MAPRRARGCRTLGLPALLLLLLLRPPATRGITCPPPMSVEHADIWVKSYSLYSRERYICNSGFKRKAGTSSLTECVLNKATNVAHWTTPSLKCIRD

SEQ ID NO: 12 - protein, 146 aa, Homo sapiens
MAPRRARGCRTLGLPALLLLLLLRPPATRGITCPPPMSVEHADIWVKSYSLYSRERYICNSGFKRKAGTSSLTECVLNKATNVAHWTTPSLKCIRDGGGGSGGGGSGGGGSEVSALEKEVSALEKEVSALEKEVSALEKEVSALEK

SEQ ID NO: 13 - protein, 403 aa, Homo sapiens
MRLAGRQVPEQRSPPPPGLGSARPGSPAVSCGAAAMAPRRARGCRTLGLPALLLLLLLRPPATRDARDRLAVLAGRSRISESFNHEVQTHEACVRLRTMENCPQCHHHRTSRQQAGITCPPPMSVEHADIWVKSYSLYSRERYICNSGFKRKAGTSSLTECVLNKATNVAHWTTPSLKCIRDPALVHQRPAPPSTVTTAGVTPQPESLSPSGKEPAASSPSSNNTAATTAAIVPGSQLMPSKSPSTGTTEISSHESSHGTPSQTTAKNWELTASASHQPPGVYPQGHSDTTVAISTSTVLLCGLSAVSLLACYLKSRQTPPLASVEMEAMEALPVTWGTSSRDEDLENCSHHLGGGGSGGGGSGGGGSEVSALEKEVSALEKEVSALEKEVSALEKEVSALEK

SEQ ID NO: 14 - protein, 317 aa, Homo sapiens
MAPRRARGCRTLGLPALLLLLLLRPPATRGITCPPPMSVEHADIWVKSYSLYSRERYICNSGFKRKAGTSSLTECVLNKATNVAHWTTPSLKCIRDPALVHQRPAPPSTVTTAGVTPQPESLSPSGKEPAASSPSSNNTAATTAAIVPGSQLMPSKSPSTGTTEISSHESSHGTPSQTTAKNWELTASASHQPPGVYPQGHSDTTVAISTSTVLLCGLSAVSLLACYLKSRQTPPLASVEMEAMEALPVTWGTSSRDEDLENCSHHLGGGGSGGGGSGGGGSEVSALEKEVSALEKEVSALEKEVSALEKEVSALEK

SEQ ID NO: 15 - protein, 215 aa, Homo sapiens
MRISKPHLRSISIQCYLCLLLNSHFLTEAGIHVFILGCFSAGLPKTEANWVNVISDLKKIEDLIQSMHIDATLYTESDVHPSCKVTAMKCFLLELQVISLESGDASIHDTVENLIILANNSLSSNGNVTESGCKECEELEEKNIKEFLQSFVHIVQMFINTSGGGGSGGGGSGGGGSCGGKVSALKEKVSALKEKVSALKEKVSALKEKVSALKE

SEQ ID NO: 16 - protein, 14 aa, Homo sapiens
TAHPSPSPRSAGQF

SEQ ID NO: 17 - protein, 10 aa, Homo sapiens
EYRMSPSNQT

SEQ ID NO: 18 - protein, 10 aa, Homo sapiens
YYRMSPSNQT

SEQ ID NO: 19 - protein, 14 aa, Mus musculus
TRYPSPSPKPEGRF

SEQ ID NO: 20 - protein, 10 aa, Homo sapiens
WNRLSPSNQT

SEQ ID NO: 21 - protein, 14 aa, Homo sapiens
TAHPSPSPRSAGQA

SEQ ID NO: 22 - protein, 14 aa, Homo sapiens
TAHPSPSPRSAGQR

SEQ ID NO: 23 - protein, 14 aa, Homo sapiens
TAHPSPSPRSAGQN

SEQ ID NO: 24 - protein, 14 aa, Homo sapiens
TAHPSPSPRSAGQD

SEQ ID NO: 25 - protein, 14 aa, Homo sapiens
TAHPSPSPRSAGQC

SEQ ID NO: 26 - protein, 14 aa, Homo sapiens
TAHPSPSPRSAGQQ

SEQ ID NO: 27 - protein, 14 aa, Homo sapiens
TAHPSPSPRSAGQE

SEQ ID NO: 28 - protein, 14 aa, Homo sapiens
TAHPSPSPRSAGQG

SEQ ID NO: 29 - protein, 14 aa, Homo sapiens
TAHPSPSPRSAGQH

SEQ ID NO: 30 - protein, 14 aa, Homo sapiens
TAHPSPSPRSAGQI

SEQ ID NO: 31 - protein, 14 aa, Homo sapiens
TAHPSPSPRSAGQL

SEQ ID NO: 32 - protein, 14 aa, Homo sapiens
TAHPSPSPRSAGQK

SEQ ID NO: 33 - protein, 14 aa, Homo sapiens
TAHPSPSPRSAGQM

SEQ ID NO: 34 - protein, 14 aa, Homo sapiens
TAHPSPSPRSAGQF

SEQ ID NO: 35 - protein, 14 aa, Homo sapiens
TAHPSPSPRSAGQP

SEQ ID NO: 36 - protein, 14 aa, Homo sapiens
TAHPSPSPRSAGQS

SEQ ID NO: 37 - protein, 14 aa, Homo sapiens
TAHPSPSPRSAGQT

SEQ ID NO: 38 - protein, 14 aa, Homo sapiens
TAHPSPSPRSAGQW

SEQ ID NO: 39 - protein, 14 aa, Homo sapiens
TAHPSPSPRSAGQY

SEQ ID NO: 40 - protein, 14 aa, Homo sapiens
TAHPSPSPRSAGQV

SEQ ID NO: 41 - protein, 14 aa, Homo sapiens
TAHPSPSPRSAGAF

SEQ ID NO: 42 - protein, 14 aa, Homo sapiens
TAHPSPSPRSAGRF

SEQ ID NO: 43 - protein, 14 aa, Homo sapiens
TAHPSPSPRSAGNF

SEQ ID NO: 44 - protein, 14 aa, Homo sapiens
TAHPSPSPRSAGDF

SEQ ID NO: 45 - protein, 14 aa, Homo sapiens
TAHPSPSPRSAGCF

SEQ ID NO: 46 - protein, 14 aa, Homo sapiens
TAHPSPSPRSAGQF

SEQ ID NO: 47 - protein, 14 aa, Homo sapiens
TAHPSPSPRSAGEF

SEQ ID NO: 48 - protein, 14 aa, Homo sapiens
TAHPSPSPRSAGGF

SEQ ID NO: 49 - protein, 14 aa, Homo sapiens
TAHPSPSPRSAGHF

SEQ ID NO: 50 - protein, 14 aa, Homo sapiens
TAHPSPSPRSAGIF

SEQ ID NO: 51 - protein, 14 aa, Homo sapiens
TAHPSPSPRSAGLF

SEQ ID NO: 52 - protein, 14 aa, Homo sapiens
TAHPSPSPRSAGKF

SEQ ID NO: 53 - protein, 14 aa, Homo sapiens
TAHPSPSPRSAGMF

SEQ ID NO: 54 - protein, 14 aa, Homo sapiens
TAHPSPSPRSAGFF

SEQ ID NO: 55 - protein, 14 aa, Homo sapiens
TAHPSPSPRSAGPF

SEQ ID NO: 56 - protein, 14 aa, Homo sapiens
TAHPSPSPRSAGSF

SEQ ID NO: 57 - protein, 14 aa, Homo sapiens
TAHPSPSPRSAGTF

SEQ ID NO: 58 - protein, 14 aa, Homo sapiens
TAHPSPSPRSAGWF

SEQ ID NO: 59 - protein, 14 aa, Homo sapiens
TAHPSPSPRSAGYF

SEQ ID NO: 60 - protein, 14 aa, Homo sapiens
TAHPSPSPRSAGVF

SEQ ID NO: 61 - protein, 14 aa, Homo sapiens
TAHPSPSPRSAAQF

SEQ ID NO: 62 - protein, 14 aa, Homo sapiens
TAHPSPSPRSARQF

SEQ ID NO: 63 - protein, 14 aa, Homo sapiens
TAHPSPSPRSANQF

SEQ ID NO: 64 - protein, 14 aa, Homo sapiens
TAHPSPSPRSADQF

SEQ ID NO: 65 - protein, 14 aa, Homo sapiens
TAHPSPSPRSACQF

SEQ ID NO: 66 - protein, 14 aa, Homo sapiens
TAHPSPSPRSAQQF

SEQ ID NO: 67 - protein, 14 aa, Homo sapiens
TAHPSPSPRSAEQF

SEQ ID NO: 68 - protein, 14 aa, Homo sapiens
TAHPSPSPRSAGQF

SEQ ID NO: 69 - protein, 14 aa, Homo sapiens
TAHPSPSPRSAHQF

SEQ ID NO: 70 - protein, 14 aa, Homo sapiens
TAHPSPSPRSAIQF

SEQ ID NO: 71 - protein, 14 aa, Homo sapiens
TAHPSPSPRSALQF

SEQ ID NO: 72 - protein, 14 aa, Homo sapiens
TAHPSPSPRSAKQF

SEQ ID NO: 73 - protein, 14 aa, Homo sapiens
TAHPSPSPRSAMQF

SEQ ID NO: 74 - protein, 14 aa, Homo sapiens
TAHPSPSPRSAFQF

SEQ ID NO: 75 - protein, 14 aa, Homo sapiens
TAHPSPSPRSAPQF

SEQ ID NO: 76 - protein, 14 aa, Homo sapiens
TAHPSPSPRSASQF

SEQ ID NO: 77 - protein, 14 aa, Homo sapiens
TAHPSPSPRSATQF

SEQ ID NO: 78 - protein, 14 aa, Homo sapiens
TAHPSPSPRSAWQF

SEQ ID NO: 79 - protein, 14 aa, Homo sapiens
TAHPSPSPRSAYQF

SEQ ID NO: 80 - protein, 14 aa, Homo sapiens
TAHPSPSPRSAVQF

SEQ ID NO: 81 - protein, 14 aa, Homo sapiens
TAHPSPSPRSAGQF

SEQ ID NO: 82 - protein, 14 aa, Homo sapiens
TAHPSPSPRSRGQF

SEQ ID NO: 83 - protein, 14 aa, Homo sapiens
TAHPSPSPRSNGQF

SEQ ID NO: 84 - protein, 14 aa, Homo sapiens
TAHPSPSPRSDGQF

SEQ ID NO: 85 - protein, 14 aa, Homo sapiens
TAHPSPSPRSCGQF

SEQ ID NO: 86 - protein, 14 aa, Homo sapiens
TAHPSPSPRSQGQF

SEQ ID NO: 87 - protein, 14 aa, Homo sapiens
TAHPSPSPRSEGQF

SEQ ID NO: 88 - protein, 14 aa, Homo sapiens
TAHPSPSPRSGGQF

SEQ ID NO: 89 - protein, 14 aa, Homo sapiens
TAHPSPSPRSHGQF

SEQ ID NO: 90 - protein, 14 aa, Homo sapiens
TAHPSPSPRSIGQF

SEQ ID NO: 91 - protein, 14 aa, Homo sapiens
TAHPSPSPRSLGQF

SEQ ID NO: 92 - protein, 14 aa, Homo sapiens
TAHPSPSPRSKGQF

SEQ ID NO: 93 - protein, 14 aa, Homo sapiens
TAHPSPSPRSMGQF

SEQ ID NO: 94 - protein, 14 aa, Homo sapiens
TAHPSPSPRSFGQF

SEQ ID NO: 95 - protein, 14 aa, Homo sapiens
TAHPSPSPRSPGQF

SEQ ID NO: 96 - protein, 14 aa, Homo sapiens
TAHPSPSPRSSGQF

SEQ ID NO: 97 - protein, 14 aa, Homo sapiens
TAHPSPSPRSTGQF

SEQ ID NO: 98 - protein, 14 aa, Homo sapiens
TAHPSPSPRSWGQF

SEQ ID NO: 99 - protein, 14 aa, Homo sapiens
TAHPSPSPRSYGQF

SEQ ID NO: 100 - protein, 14 aa, Homo sapiens
TAHPSPSPRSVGQF

SEQ ID NO: 101 - protein, 14 aa, Homo sapiens
TAHPSPSPRAAGQF

SEQ ID NO: 102 - protein, 14 aa, Homo sapiens
TAHPSPSPRRAGQF

SEQ ID NO: 103 - protein, 14 aa, Homo sapiens
TAHPSPSPRNAGQF

SEQ ID NO: 104 - protein, 14 aa, Homo sapiens
TAHPSPSPRDAGQF

SEQ ID NO: 105 - protein, 14 aa, Homo sapiens
TAHPSPSPRCAGQF

SEQ ID NO: 106 - protein, 14 aa, Homo sapiens
TAHPSPSPRQAGQF

SEQ ID NO: 107 - protein, 14 aa, Homo sapiens
TAHPSPSPREAGQF

SEQ ID NO: 108 - protein, 14 aa, Homo sapiens
TAHPSPSPRGAGQF

SEQ ID NO: 109 - protein, 14 aa, Homo sapiens
TAHPSPSPRHAGQF

SEQ ID NO: 110 - protein, 14 aa, Homo sapiens
TAHPSPSPRIAGQF

SEQ ID NO: 111 - protein, 14 aa, Homo sapiens
TAHPSPSPRLAGQF

SEQ ID NO: 112 - protein, 14 aa, Homo sapiens
TAHPSPSPRKAGQF

SEQ ID NO: 113 - protein, 14 aa, Homo sapiens
TAHPSPSPRMAGQF

SEQ ID NO: 114 - protein, 14 aa, Homo sapiens
TAHPSPSPRFAGQF

SEQ ID NO: 115 - protein, 14 aa, Homo sapiens
TAHPSPSPRPAGQF

SEQ ID NO: 116 - protein, 14 aa, Homo sapiens
TAHPSPSPRSAGQF

SEQ ID NO: 117 - protein, 14 aa, Homo sapiens
TAHPSPSPRTAGQF

SEQ ID NO: 118 - protein, 14 aa, Homo sapiens
TAHPSPSPRWAGQF

SEQ ID NO: 119 - protein, 14 aa, Homo sapiens
TAHPSPSPRYAGQF

SEQ ID NO: 120 - protein, 14 aa, Homo sapiens
TAHPSPSPRVAGQF

SEQ ID NO: 121 - protein, 14 aa, Homo sapiens
TAHPSPSPASAGQF

SEQ ID NO: 122 - protein, 14 aa, Homo sapiens
TAHPSPSPRSAGQF

SEQ ID NO: 123 - protein, 14 aa, Homo sapiens
TAHPSPSPNSAGQF

SEQ ID NO: 124 - protein, 14 aa, Homo sapiens
TAHPSPSPDSAGQF

SEQ ID NO: 125 - protein, 14 aa, Homo sapiens
TAHPSPSPCSAGQF

SEQ ID NO: 126 - protein, 14 aa, Homo sapiens
TAHPSPSPQSAGQF

SEQ ID NO: 127 - protein, 14 aa, Homo sapiens
TAHPSPSPESAGQF

SEQ ID NO: 128 - protein, 14 aa, Homo sapiens
TAHPSPSPGSAGQF

SEQ ID NO: 129 - protein, 14 aa, Homo sapiens
TAHPSPSPHSAGQF

SEQ ID NO: 130 - protein, 14 aa, Homo sapiens
TAHPSPSPISAGQF

SEQ ID NO: 131 - protein, 14 aa, Homo sapiens
TAHPSPSPLSAGQF

SEQ ID NO: 132 - protein, 14 aa, Homo sapiens
TAHPSPSPKSAGQF

SEQ ID NO: 133 - protein, 14 aa, Homo sapiens
TAHPSPSPMSAGQF

SEQ ID NO: 134 - protein, 14 aa, Homo sapiens
TAHPSPSPFSAGQF

SEQ ID NO: 135 - protein, 14 aa, Homo sapiens
TAHPSPSPPSAGQF

SEQ ID NO: 136 - protein, 14 aa, Homo sapiens
TAHPSPSPSSAGQF

SEQ ID NO: 137 - protein, 14 aa, Homo sapiens
TAHPSPSPTSAGQF

SEQ ID NO: 138 - protein, 14 aa, Homo sapiens
TAHPSPSPWSAGQF

SEQ ID NO: 139 - protein, 14 aa, Homo sapiens
TAHPSPSPYSAGQF

SEQ ID NO: 140 - protein, 14 aa, Homo sapiens
TAHPSPSPVSAGQF

SEQ ID NO: 141 - protein, 14 aa, Homo sapiens
TAHPSPSARSAGQF

SEQ ID NO: 142 - protein, 14 aa, Homo sapiens
TAHPSPSRRSAGQF

SEQ ID NO: 143 - protein, 14 aa, Homo sapiens
TAHPSPSNRSAGQF

SEQ ID NO: 144 - protein, 14 aa, Homo sapiens
TAHPSPSDRSAGQF

SEQ ID NO: 145 - protein, 14 aa, Homo sapiens
TAHPSPSCRSAGQF

SEQ ID NO: 146 - protein, 14 aa, Homo sapiens
TAHPSPSQRSAGQF

SEQ ID NO: 147 - protein, 14 aa, Homo sapiens
TAHPSPSERSAGQF

SEQ ID NO: 148 - protein, 14 aa, Homo sapiens
TAHPSPSGRSAGQF

SEQ ID NO: 149 - protein, 14 aa, Homo sapiens
TAHPSPSHRSAGQF

SEQ ID NO: 150 - protein, 14 aa, Homo sapiens
TAHPSPSIRSAGQF

SEQ ID NO: 151 - protein, 14 aa, Homo sapiens
TAHPSPSLRSAGQF

SEQ ID NO: 152 - protein, 14 aa, Homo sapiens
TAHPSPSKRSAGQF

SEQ ID NO: 153 - protein, 14 aa, Homo sapiens
TAHPSPSMRSAGQF

SEQ ID NO: 154 - protein, 14 aa, Homo sapiens
TAHPSPSFRSAGQF

SEQ ID NO: 155 - protein, 14 aa, Homo sapiens
TAHPSPSPRSAGQF

SEQ ID NO: 156 - protein, 14 aa, Homo sapiens
TAHPSPSSRSAGQF

SEQ ID NO: 157 - protein, 14 aa, Homo sapiens
TAHPSPSTRSAGQF

SEQ ID NO: 158 - protein, 14 aa, Homo sapiens
TAHPSPSWRSAGQF

SEQ ID NO: 159 - protein, 14 aa, Homo sapiens
TAHPSPSYRSAGQF

SEQ ID NO: 160 - protein, 14 aa, Homo sapiens
TAHPSPSVRSAGQF

SEQ ID NO: 161 - protein, 14 aa, Homo sapiens
TAHPSPAPRSAGQF

SEQ ID NO: 162 - protein, 14 aa, Homo sapiens
TAHPSPRPRSAGQF

SEQ ID NO: 163 - protein, 14 aa, Homo sapiens
TAHPSPNPRSAGQF

SEQ ID NO: 164 - protein, 14 aa, Homo sapiens
TAHPSPDPRSAGQF

SEQ ID NO: 165 - protein, 14 aa, Homo sapiens
TAHPSPCPRSAGQF

SEQ ID NO: 166 - protein, 14 aa, Homo sapiens
TAHPSPEPRSAGQF

SEQ ID NO: 167 - protein, 14 aa, Homo sapiens
TAHPSPQPRSAGQF

SEQ ID NO: 168 - protein, 14 aa, Homo sapiens
TAHPSPGPRSAGQF

SEQ ID NO: 169 - protein, 14 aa, Homo sapiens
TAHPSPHPRSAGQF

SEQ ID NO: 170 - protein, 14 aa, Homo sapiens
TAHPSPIPRSAGQF

SEQ ID NO: 171 - protein, 14 aa, Homo sapiens
TAHPSPLPRSAGQF

SEQ ID NO: 172 - protein, 14 aa, Homo sapiens
TAHPSPKPRSAGQF

SEQ ID NO: 173 - protein, 14 aa, Homo sapiens
TAHPSPMPRSAGQF

SEQ ID NO: 174 - protein, 14 aa, Homo sapiens
TAHPSPFPRSAGQF

SEQ ID NO: 175 - protein, 14 aa, Homo sapiens
TAHPSPPPRSAGQF

SEQ ID NO: 176 - protein, 14 aa, Homo sapiens
TAHPSPSPRSAGQF

SEQ ID NO: 177 - protein, 14 aa, Homo sapiens
TAHPSPTPRSAGQF

SEQ ID NO: 178 - protein, 14 aa, Homo sapiens
TAHPSPWPRSAGQF

SEQ ID NO: 179 - protein, 14 aa, Homo sapiens
TAHPSPYPRSAGQF

SEQ ID NO: 180 - protein, 14 aa, Homo sapiens
TAHPSPVPRSAGQF

SEQ ID NO: 181 - protein, 14 aa, Homo sapiens
TAHPSASPRSAGQF

SEQ ID NO: 182 - protein, 14 aa, Homo sapiens
TAHPSRSPRSAGQF

SEQ ID NO: 183 - protein, 14 aa, Homo sapiens
TAHPSNSPRSAGQF

SEQ ID NO: 184 - protein, 14 aa, Homo sapiens
TAHPSDSPRSAGQF

SEQ ID NO: 185 - protein, 14 aa, Homo sapiens
TAHPSCSPRSAGQF

SEQ ID NO: 186 - protein, 14 aa, Homo sapiens
TAHPSQSPRSAGQF

SEQ ID NO: 187 - protein, 14 aa, Homo sapiens
TAHPSESPRSAGQF

SEQ ID NO: 188 - protein, 14 aa, Homo sapiens
TAHPSGSPRSAGQF

SEQ ID NO: 189 - protein, 14 aa, Homo sapiens
TAHPSHSPRSAGQF

SEQ ID NO: 190 - protein, 14 aa, Homo sapiens
TAHPSISPRSAGQF

SEQ ID NO: 191 - protein, 14 aa, Homo sapiens
TAHPSLSPRSAGQF

SEQ ID NO: 192 - protein, 14 aa, Homo sapiens
TAHPSKSPRSAGQF

SEQ ID NO: 193 - protein, 14 aa, Homo sapiens
TAHPSMSPRSAGQF

SEQ ID NO: 194 - protein, 14 aa, Homo sapiens
TAHPSFSPRSAGQF

SEQ ID NO: 195 - protein, 14 aa, Homo sapiens
TAHPSPSPRSAGQF

SEQ ID NO: 196 - protein, 14 aa, Homo sapiens
TAHPSSSPRSAGQF

SEQ ID NO: 197 - protein, 14 aa, Homo sapiens
TAHPSTSPRSAGQF

SEQ ID NO: 198 - protein, 14 aa, Homo sapiens
TAHPSWSPRSAGQF

SEQ ID NO: 199 - protein, 14 aa, Homo sapiens
TAHPSYSPRSAGQF

SEQ ID NO: 200 - protein, 14 aa, Homo sapiens
TAHPSVSPRSAGQF

SEQ ID NO: 201 - protein, 14 aa, Homo sapiens
TAHPAPSPRSAGQF

SEQ ID NO: 202 - protein, 14 aa, Homo sapiens
TAHPRPSPRSAGQF

SEQ ID NO: 203 - protein, 14 aa, Homo sapiens
TAHPNPSPRSAGQF

SEQ ID NO: 204 - protein, 14 aa, Homo sapiens
TAHPDPSPRSAGQF

SEQ ID NO: 205 - protein, 14 aa, Homo sapiens
TAHPCPSPRSAGQF

SEQ ID NO: 206 - protein, 14 aa, Homo sapiens
TAHPQPSPRSAGQF

SEQ ID NO: 207 - protein, 14 aa, Homo sapiens
TAHPEPSPRSAGQF

SEQ ID NO: 208 - protein, 14 aa, Homo sapiens
TAHPGPSPRSAGQF

SEQ ID NO: 209 - protein, 14 aa, Homo sapiens
TAHPHPSPRSAGQF

SEQ ID NO: 210 - protein, 14 aa, Homo sapiens
TAHPIPSPRSAGQF

SEQ ID NO: 211 - protein, 14 aa, Homo sapiens
TAHPLPSPRSAGQF

SEQ ID NO: 212 - protein, 14 aa, Homo sapiens
TAHPKPSPRSAGQF

SEQ ID NO: 213 - protein, 14 aa, Homo sapiens
TAHPMPSPRSAGQF

SEQ ID NO: 214 - protein, 14 aa, Homo sapiens
TAHPFPSPRSAGQF

SEQ ID NO: 215 - protein, 14 aa, Homo sapiens
TAHPPPSPRSAGQF

SEQ ID NO: 216 - protein, 14 aa, Homo sapiens
TAHPSPSPRSAGQF

SEQ ID NO: 217 - protein, 14 aa, Homo sapiens
TAHPTPSPRSAGQF

SEQ ID NO: 218 - protein, 14 aa, Homo sapiens
TAHPWPSPRSAGQF

SEQ ID NO: 219 - protein, 14 aa, Homo sapiens
TAHPYPSPRSAGQF

SEQ ID NO: 220 - protein, 14 aa, Homo sapiens
TAHPVPSPRSAGQF

SEQ ID NO: 221 - protein, 14 aa, Homo sapiens
TAHASPSPRSAGQF

SEQ ID NO: 222 - protein, 14 aa, Homo sapiens
TAHRSPSPRSAGQF

SEQ ID NO: 223 - protein, 14 aa, Homo sapiens
TAHNSPSPRSAGQF

SEQ ID NO: 224 - protein, 14 aa, Homo sapiens
TAHDSPSPRSAGQF

SEQ ID NO: 225 - protein, 14 aa, Homo sapiens
TAHCSPSPRSAGQF

SEQ ID NO: 226 - protein, 14 aa, Homo sapiens
TAHQSPSPRSAGQF

SEQ ID NO: 227 - protein, 14 aa, Homo sapiens
TAHESPSPRSAGQF

SEQ ID NO: 228 - protein, 14 aa, Homo sapiens
TAHGSPSPRSAGQF

SEQ ID NO: 229 - protein, 14 aa, Homo sapiens
TAHHSPSPRSAGQF

SEQ ID NO: 230 - protein, 14 aa, Homo sapiens
TAHISPSPRSAGQF

SEQ ID NO: 231 - protein, 14 aa, Homo sapiens
TAHLSPSPRSAGQF

SEQ ID NO: 232 - protein, 14 aa, Homo sapiens
TAHKSPSPRSAGQF

SEQ ID NO: 233 - protein, 14 aa, Homo sapiens
TAHMSPSPRSAGQF

SEQ ID NO: 234 - protein, 14 aa, Homo sapiens
TAHFSPSPRSAGQF

SEQ ID NO: 235 - protein, 14 aa, Homo sapiens
TAHPSPSPRSAGQF

SEQ ID NO: 236 - protein, 14 aa, Homo sapiens
TAHSSPSPRSAGQF

SEQ ID NO: 237 - protein, 14 aa, Homo sapiens
TAHTSPSPRSAGQF

SEQ ID NO: 238 - protein, 14 aa, Homo sapiens
TAHWSPSPRSAGQF

SEQ ID NO: 239 - protein, 14 aa, Homo sapiens
TAHYSPSPRSAGQF

SEQ ID NO: 240 - protein, 14 aa, Homo sapiens
TAHVSPSPRSAGQF

SEQ ID NO: 241 - protein, 14 aa, Homo sapiens
TAAPSPSPRSAGQF

SEQ ID NO: 242 - protein, 14 aa, Homo sapiens
TARPSPSPRSAGQF

SEQ ID NO: 243 - protein, 14 aa, Homo sapiens
TANPSPSPRSAGQF

SEQ ID NO: 244 - protein, 14 aa, Homo sapiens
TADPSPSPRSAGQF

SEQ ID NO: 245 - protein, 14 aa, Homo sapiens
TACPSPSPRSAGQF

SEQ ID NO: 246 - protein, 14 aa, Homo sapiens
TAQPSPSPRSAGQF

SEQ ID NO: 247 - protein, 14 aa, Homo sapiens
TAEPSPSPRSAGQF

SEQ ID NO: 248 - protein, 14 aa, Homo sapiens
TAGPSPSPRSAGQF

SEQ ID NO: 249 - protein, 14 aa, Homo sapiens
TAHPSPSPRSAGQF

SEQ ID NO: 250 - protein, 14 aa, Homo sapiens
TAIPSPSPRSAGQF

SEQ ID NO: 251 - protein, 14 aa, Homo sapiens
TALPSPSPRSAGQF

SEQ ID NO: 252 - protein, 14 aa, Homo sapiens
TAKPSPSPRSAGQF

SEQ ID NO: 253 - protein, 14 aa, Homo sapiens
TAMPSPSPRSAGQF

SEQ ID NO: 254 - protein, 14 aa, Homo sapiens
TAFPSPSPRSAGQF

SEQ ID NO: 255 - protein, 14 aa, Homo sapiens
TAPPSPSPRSAGQF

SEQ ID NO: 256 - protein, 14 aa, Homo sapiens
TASPSPSPRSAGQF

SEQ ID NO: 257 - protein, 14 aa, Homo sapiens
TATPSPSPRSAGQF

SEQ ID NO: 258 - protein, 14 aa, Homo sapiens
TAWPSPSPRSAGQF

SEQ ID NO: 259 - protein, 14 aa, Homo sapiens
TAYPSPSPRSAGQF

SEQ ID NO: 260 - protein, 14 aa, Homo sapiens
TAVPSPSPRSAGQF

SEQ ID NO: 261 - protein, 14 aa, Homo sapiens
TAHPSPSPRSAGQF

SEQ ID NO: 262 - protein, 14 aa, Homo sapiens
TRHPSPSPRSAGQF

SEQ ID NO: 263 - protein, 14 aa, Homo sapiens
TNHPSPSPRSAGQF

SEQ ID NO: 264 - protein, 14 aa, Homo sapiens
TDHPSPSPRSAGQF

SEQ ID NO: 265 - protein, 14 aa, Homo sapiens
TCHPSPSPRSAGQF

SEQ ID NO: 266 - protein, 14 aa, Homo sapiens
TQHPSPSPRSAGQF

SEQ ID NO: 267 - protein, 14 aa, Homo sapiens
TEHPSPSPRSAGQF

SEQ ID NO: 268 - protein, 14 aa, Homo sapiens
TGHPSPSPRSAGQF

SEQ ID NO: 269 - protein, 14 aa, Homo sapiens
THHPSPSPRSAGQF

SEQ ID NO: 270 - protein, 14 aa, Homo sapiens
TIHPSPSPRSAGQF

SEQ ID NO: 271 - protein, 14 aa, Homo sapiens
TLHPSPSPRSAGQF

SEQ ID NO: 272 - protein, 14 aa, Homo sapiens
TKHPSPSPRSAGQF

SEQ ID NO: 273 - protein, 14 aa, Homo sapiens
TMHPSPSPRSAGQF

SEQ ID NO: 274 - protein, 14 aa, Homo sapiens
TFHPSPSPRSAGQF

SEQ ID NO: 275 - protein, 14 aa, Homo sapiens
TPHPSPSPRSAGQF

SEQ ID NO: 276 - protein, 14 aa, Homo sapiens
TSHPSPSPRSAGQF

SEQ ID NO: 277 - protein, 14 aa, Homo sapiens
TTHPSPSPRSAGQF

SEQ ID NO: 278 - protein, 14 aa, Homo sapiens
TWHPSPSPRSAGQF

SEQ ID NO: 279 - protein, 14 aa, Homo sapiens
TYHPSPSPRSAGQF

SEQ ID NO: 280 - protein, 14 aa, Homo sapiens
TVHPSPSPRSAGQF

SEQ ID NO: 281 - protein, 14 aa, Homo sapiens
AAHPSPSPRSAGQF

SEQ ID NO: 282 - protein, 14 aa, Homo sapiens
RAHPSPSPRSAGQF

SEQ ID NO: 283 - protein, 14 aa, Homo sapiens
NAHPSPSPRSAGQF

SEQ ID NO: 284 - protein, 14 aa, Homo sapiens
DAHPSPSPRSAGQF

SEQ ID NO: 285 - protein, 14 aa, Homo sapiens
CAHPSPSPRSAGQF

SEQ ID NO: 286 - protein, 14 aa, Homo sapiens
QAHPSPSPRSAGQF

SEQ ID NO: 287 - protein, 14 aa, Homo sapiens
EAHPSPSPRSAGQF

SEQ ID NO: 288 - protein, 14 aa, Homo sapiens
GAHPSPSPRSAGQF

SEQ ID NO: 289 - protein, 14 aa, Homo sapiens
HAHPSPSPRSAGQF

SEQ ID NO: 290 - protein, 14 aa, Homo sapiens
IAHPSPSPRSAGQF

SEQ ID NO: 291 - protein, 14 aa, Homo sapiens
LAHPSPSPRSAGQF

SEQ ID NO: 292 - protein, 14 aa, Homo sapiens
KAHPSPSPRSAGQF

SEQ ID NO: 293 - protein, 14 aa, Homo sapiens
MAHPSPSPRSAGQF

SEQ ID NO: 294 - protein, 14 aa, Homo sapiens
FAHPSPSPRSAGQF

SEQ ID NO: 295 - protein, 14 aa, Homo sapiens
PAHPSPSPRSAGQF

SEQ ID NO: 296 - protein, 14 aa, Homo sapiens
SAHPSPSPRSAGQF

SEQ ID NO: 297 - protein, 14 aa, Homo sapiens
TAHPSPSPRSAGQF

SEQ ID NO: 298 - protein, 14 aa, Homo sapiens
WAHPSPSPRSAGQF

SEQ ID NO: 299 - protein, 14 aa, Homo sapiens
YAHPSPSPRSAGQF

SEQ ID NO: 300 - protein, 14 aa, Homo sapiens
VAHPSPSPRSAGQF

SEQ ID NO: 301 - protein, 10 aa, Homo sapiens
WYRMSPSNQA

SEQ ID NO: 302 - protein, 10 aa, Homo sapiens
WYRMSPSNQR

SEQ ID NO: 303 - protein, 10 aa, Homo sapiens
WYRMSPSNQN

SEQ ID NO: 304 - protein, 10 aa, Homo sapiens
WYRMSPSNQD

SEQ ID NO: 305 - protein, 10 aa, Homo sapiens
WYRMSPSNQC

SEQ ID NO: 306 - protein, 10 aa, Homo sapiens
WYRMSPSNQQ

SEQ ID NO: 307 - protein, 10 aa, Homo sapiens
WYRMSPSNQE

SEQ ID NO: 308 - protein, 10 aa, Homo sapiens
WYRMSPSNQG

SEQ ID NO: 309 - protein, 10 aa, Homo sapiens
WYRMSPSNQH

SEQ ID NO: 310 - protein, 10 aa, Homo sapiens
WYRMSPSNQI

SEQ ID NO: 311 - protein, 10 aa, Homo sapiens
WYRMSPSNQL

SEQ ID NO: 312 - protein, 10 aa, Homo sapiens
WYRMSPSNQK

SEQ ID NO: 313 - protein, 10 aa, Homo sapiens
WYRMSPSNQM

SEQ ID NO: 314 - protein, 10 aa, Homo sapiens
WYRMSPSNQF

SEQ ID NO: 315 - protein, 10 aa, Homo sapiens
WYRMSPSNQP

SEQ ID NO: 316 - protein, 10 aa, Homo sapiens
WYRMSPSNQS

SEQ ID NO: 317 - protein, 10 aa, Homo sapiens
WYRMSPSNQT

SEQ ID NO: 318 - protein, 10 aa, Homo sapiens
WYRMSPSNQW

SEQ ID NO: 319 - protein, 10 aa, Homo sapiens
WYRMSPSNQY

SEQ ID NO: 320 - protein, 10 aa, Homo sapiens
WYRMSPSNQV

SEQ ID NO: 321 - protein, 10 aa, Homo sapiens
WYRMSPSNAT

SEQ ID NO: 322 - protein, 10 aa, Homo sapiens
WYRMSPSNRT

SEQ ID NO: 323 - protein, 10 aa, Homo sapiens
WYRMSPSNNT

SEQ ID NO: 324 - protein, 10 aa, Homo sapiens
WYRMSPSNDT

SEQ ID NO: 325 - protein, 10 aa, Homo sapiens
WYRMSPSNCT

SEQ ID NO: 326 - protein, 10 aa, Homo sapiens
WYRMSPSNQT

SEQ ID NO: 327 - protein, 10 aa, Homo sapiens
WYRMSPSNET

SEQ ID NO: 328 - protein, 10 aa, Homo sapiens
WYRMSPSNGT

SEQ ID NO: 329 - protein, 10 aa, Homo sapiens
WYRMSPSNHT

SEQ ID NO: 330 - protein, 10 aa, Homo sapiens
WYRMSPSNIT

SEQ ID NO: 331 - protein, 10 aa, Homo sapiens
WYRMSPSNLT

SEQ ID NO: 332 - protein, 10 aa, Homo sapiens
WYRMSPSNKT

SEQ ID NO: 333 - protein, 10 aa, Homo sapiens
WYRMSPSNMT

SEQ ID NO: 334 - protein, 10 aa, Homo sapiens
WYRMSPSNFT

SEQ ID NO: 335 - protein, 10 aa, Homo sapiens
WYRMSPSNPT

SEQ ID NO: 336 - protein, 10 aa, Homo sapiens
WYRMSPSNST

SEQ ID NO: 337 - protein, 10 aa, Homo sapiens
WYRMSPSNTT

SEQ ID NO: 338 - protein, 10 aa, Homo sapiens
WYRMSPSNWT

SEQ ID NO: 339 - protein, 10 aa, Homo sapiens
WYRMSPSNYT

SEQ ID NO: 340 - protein, 10 aa, Homo sapiens
WYRMSPSNVT

SEQ ID NO: 341 - protein, 10 aa, Homo sapiens
WYRMSPSAQT

SEQ ID NO: 342 - protein, 10 aa, Homo sapiens
WYRMSPSRQT

SEQ ID NO: 343 - protein, 10 aa, Homo sapiens
WYRMSPSNQT

SEQ ID NO: 344 - protein, 10 aa, Homo sapiens
WYRMSPSDQT

SEQ ID NO: 345 - protein, 10 aa, Homo sapiens
WYRMSPSCQT

SEQ ID NO: 346 - protein, 10 aa, Homo sapiens
WYRMSPSQQT

SEQ ID NO: 347 - protein, 10 aa, Homo sapiens
WYRMSPSEQT

SEQ ID NO: 348 - protein, 10 aa, Homo sapiens
WYRMSPSGQT

SEQ ID NO: 349 - protein, 10 aa, Homo sapiens
WYRMSPSHQT

SEQ ID NO: 350 - protein, 10 aa, Homo sapiens
WYRMSPSIQT

SEQ ID NO: 351 - protein, 10 aa, Homo sapiens
WYRMSPSLQT

SEQ ID NO: 352 - protein, 10 aa, Homo sapiens
WYRMSPSKQT

SEQ ID NO: 353 - protein, 10 aa, Homo sapiens
WYRMSPSMQT

SEQ ID NO: 354 - protein, 10 aa, Homo sapiens
WYRMSPSFQT

SEQ ID NO: 355 - protein, 10 aa, Homo sapiens
WYRMSPSPQT

SEQ ID NO: 356 - protein, 10 aa, Homo sapiens
WYRMSPSSQT

SEQ ID NO: 357 - protein, 10 aa, Homo sapiens
WYRMSPSTQT

SEQ ID NO: 358 - protein, 10 aa, Homo sapiens
WYRMSPSWQT

SEQ ID NO: 359 - protein, 10 aa, Homo sapiens
WYRMSPSYQT

SEQ ID NO: 360 - protein, 10 aa, Homo sapiens
WYRMSPSVQT

SEQ ID NO: 361 - protein, 10 aa, Homo sapiens
WYRMSPANQT

SEQ ID NO: 362 - protein, 10 aa, Homo sapiens
WYRMSPRNQT

SEQ ID NO: 363 - protein, 10 aa, Homo sapiens
WYRMSPNNQT

SEQ ID NO: 364 - protein, 10 aa, Homo sapiens
WYRMSPDNQT

SEQ ID NO: 365 - protein, 10 aa, Homo sapiens
WYRMSPCNQT

SEQ ID NO: 366 - protein, 10 aa, Homo sapiens
WYRMSPQNQT

SEQ ID NO: 367 - protein, 10 aa, Homo sapiens
WYRMSPENQT

SEQ ID NO: 368 - protein, 10 aa, Homo sapiens
WYRMSPGNQT

SEQ ID NO: 369 - protein, 10 aa, Homo sapiens
WYRMSPHNQT

SEQ ID NO: 370 - protein, 10 aa, Homo sapiens
WYRMSPINQT

SEQ ID NO: 371 - protein, 10 aa, Homo sapiens
WYRMSPLNQT

SEQ ID NO: 372 - protein, 10 aa, Homo sapiens
WYRMSPKNQT

SEQ ID NO: 373 - protein, 10 aa, Homo sapiens
WYRMSPMNQT

SEQ ID NO: 374 - protein, 10 aa, Homo sapiens
WYRMSPFNQT

SEQ ID NO: 375 - protein, 10 aa, Homo sapiens
WYRMSPPNQT

SEQ ID NO: 376 - protein, 10 aa, Homo sapiens
WYRMSPSNQT

SEQ ID NO: 377 - protein, 10 aa, Homo sapiens
WYRMSPTNQT

SEQ ID NO: 378 - protein, 10 aa, Homo sapiens
WYRMSPWNQT

SEQ ID NO: 379 - protein, 10 aa, Homo sapiens
WYRMSPYNQT

SEQ ID NO: 380 - protein, 10 aa, Homo sapiens
WYRMSPVNQT

SEQ ID NO: 381 - protein, 10 aa, Homo sapiens
WYRMSASNQT

SEQ ID NO: 382 - protein, 10 aa, Homo sapiens
WYRMSRSNQT

SEQ ID NO: 383 - protein, 10 aa, Homo sapiens
WYRMSNSNQT

SEQ ID NO: 384 - protein, 10 aa, Homo sapiens
WYRMSDSNQT

SEQ ID NO: 385 - protein, 10 aa, Homo sapiens
WYRMSCSNQT

SEQ ID NO: 386 - protein, 10 aa, Homo sapiens
WYRMSQSNQT

SEQ ID NO: 387 - protein, 10 aa, Homo sapiens
WYRMSESNQT

SEQ ID NO: 388 - protein, 10 aa, Homo sapiens
WYRMSGSNQT

SEQ ID NO: 389 - protein, 10 aa, Homo sapiens
WYRMSHSNQT

SEQ ID NO: 390 - protein, 10 aa, Homo sapiens
WYRMSISNQT

SEQ ID NO: 391 - protein, 10 aa, Homo sapiens
WYRMSLSNQT

SEQ ID NO: 392 - protein, 10 aa, Homo sapiens
WYRMSKSNQT

SEQ ID NO: 393 - protein, 10 aa, Homo sapiens
WYRMSMSNQT

SEQ ID NO: 394 - protein, 10 aa, Homo sapiens
WYRMSFSNQT

SEQ ID NO: 395 - protein, 10 aa, Homo sapiens
WYRMSPSNQT

SEQ ID NO: 396 - protein, 10 aa, Homo sapiens
WYRMSSSNQT

SEQ ID NO: 397 - protein, 10 aa, Homo sapiens
WYRMSTSNQT

SEQ ID NO: 398 - protein, 10 aa, Homo sapiens
WYRMSWSNQT

SEQ ID NO: 399 - protein, 10 aa, Homo sapiens
WYRMSYSNQT

SEQ ID NO: 400 - protein, 10 aa, Homo sapiens
WYRMSVSNQT

SEQ ID NO: 401 - protein, 10 aa, Homo sapiens
WYRMAPSNQT

SEQ ID NO: 402 - protein, 10 aa, Homo sapiens
WYRMRPSNQT

SEQ ID NO: 403 - protein, 10 aa, Homo sapiens
WYRMNPSNQT

SEQ ID NO: 404 - protein, 10 aa, Homo sapiens
WYRMDPSNQT

SEQ ID NO: 405 - protein, 10 aa, Homo sapiens
WYRMCPSNQT

SEQ ID NO: 406 - protein, 10 aa, Homo sapiens
WYRMQPSNQT

SEQ ID NO: 407 - protein, 10 aa, Homo sapiens
WYRMEPSNQT

SEQ ID NO: 408 - protein, 10 aa, Homo sapiens
WYRMGPSNQT

SEQ ID NO: 409 - protein, 10 aa, Homo sapiens
WYRMHPSNQT

SEQ ID NO: 410 - protein, 10 aa, Homo sapiens
WYRMIPSNQT

SEQ ID NO: 411 - protein, 10 aa, Homo sapiens
WYRMLPSNQT

SEQ ID NO: 412 - protein, 10 aa, Homo sapiens
WYRMKPSNQT

SEQ ID NO: 413 - protein, 10 aa, Homo sapiens
WYRMMPSNQT

SEQ ID NO: 414 - protein, 10 aa, Homo sapiens
WYRMFPSNQT

SEQ ID NO: 415 - protein, 10 aa, Homo sapiens
WYRMPPSNQT

SEQ ID NO: 416 - protein, 10 aa, Homo sapiens
WYRMSPSNQT

SEQ ID NO: 417 - protein, 10 aa, Homo sapiens
WYRMTPSNQT

SEQ ID NO: 418 - protein, 10 aa, Homo sapiens
WYRMWPSNQT

SEQ ID NO: 419 - protein, 10 aa, Homo sapiens
WYRMYPSNQT

SEQ ID NO: 420 - protein, 10 aa, Homo sapiens
WYRMVPSNQT

SEQ ID NO: 421 - protein, 10 aa, Homo sapiens
WYRASPSNQT

SEQ ID NO: 422 - protein, 10 aa, Homo sapiens
WYRRSPSNQT

SEQ ID NO: 423 - protein, 10 aa, Homo sapiens
WYRNSPSNQT

SEQ ID NO: 424 - protein, 10 aa, Homo sapiens
WYRDSPSNQT

SEQ ID NO: 425 - protein, 10 aa, Homo sapiens
WYRCSPSNQT

SEQ ID NO: 426 - protein, 10 aa, Homo sapiens
WYRQSPSNQT

SEQ ID NO: 427 - protein, 10 aa, Homo sapiens
WYRESPSNQT

SEQ ID NO: 428 - protein, 10 aa, Homo sapiens
WYRGSPSNQT

SEQ ID NO: 429 - protein, 10 aa, Homo sapiens
WYRHSPSNQT

SEQ ID NO: 430 - protein, 10 aa, Homo sapiens
WYRISPSNQT

SEQ ID NO: 431 - protein, 10 aa, Homo sapiens
WYRLSPSNQT

SEQ ID NO: 432 - protein, 10 aa, Homo sapiens
WYRKSPSNQT

SEQ ID NO: 433 - protein, 10 aa, Homo sapiens
WYRMSPSNQT

SEQ ID NO: 434 - protein, 10 aa, Homo sapiens
WYRFSPSNQT

SEQ ID NO: 435 - protein, 10 aa, Homo sapiens
WYRPSPSNQT

SEQ ID NO: 436 - protein, 10 aa, Homo sapiens
WYRSSPSNQT

SEQ ID NO: 437 - protein, 10 aa, Homo sapiens
WYRTSPSNQT

SEQ ID NO: 438 - protein, 10 aa, Homo sapiens
WYRWSPSNQT

SEQ ID NO: 439 - protein, 10 aa, Homo sapiens
WYRYSPSNQT

SEQ ID NO: 440 - protein, 10 aa, Homo sapiens
WYRVSPSNQT

SEQ ID NO: 441 - protein, 10 aa, Homo sapiens
WYAMSPSNQT

SEQ ID NO: 442 - protein, 10 aa, Homo sapiens
WYRMSPSNQT

SEQ ID NO: 443 - protein, 10 aa, Homo sapiens
WYNMSPSNQT

SEQ ID NO: 444 - protein, 10 aa, Homo sapiens
WYDMSPSNQT

SEQ ID NO: 445 - protein, 10 aa, Homo sapiens
WYCMSPSNQT

SEQ ID NO: 446 - protein, 10 aa, Homo sapiens
WYQMSPSNQT

SEQ ID NO: 447 - protein, 10 aa, Homo sapiens
WYEMSPSNQT

SEQ ID NO: 448 - protein, 10 aa, Homo sapiens
WYGMSPSNQT

SEQ ID NO: 449 - protein, 10 aa, Homo sapiens
WYHMSPSNQT

SEQ ID NO: 450 - protein, 10 aa, Homo sapiens
WYIMSPSNQT

SEQ ID NO: 451 - protein, 10 aa, Homo sapiens
WYLMSPSNQT

SEQ ID NO: 452 - protein, 10 aa, Homo sapiens
WYKMSPSNQT

SEQ ID NO: 453 - protein, 10 aa, Homo sapiens
WYMMSPSNQT

SEQ ID NO: 454 - protein, 10 aa, Homo sapiens
WYFMSPSNQT

SEQ ID NO: 455 - protein, 10 aa, Homo sapiens
WYPMSPSNQT

SEQ ID NO: 456 - protein, 10 aa, Homo sapiens
WYSMSPSNQT

SEQ ID NO: 457 - protein, 10 aa, Homo sapiens
WYTMSPSNQT

SEQ ID NO: 458 - protein, 10 aa, Homo sapiens
WYWMSPSNQT

SEQ ID NO: 459 - protein, 10 aa, Homo sapiens
WYYMSPSNQT

SEQ ID NO: 460 - protein, 10 aa, Homo sapiens
WYVMSPSNQT

SEQ ID NO: 461 - protein, 10 aa, Homo sapiens
WARMSPSNQT

SEQ ID NO: 462 - protein, 10 aa, Homo sapiens
WRRMSPSNQT

SEQ ID NO: 463 - protein, 10 aa, Homo sapiens
WNRMSPSNQT

SEQ ID NO: 464 - protein, 10 aa, Homo sapiens
WDRMSPSNQT

SEQ ID NO: 465 - protein, 10 aa, Homo sapiens
WCRMSPSNQT

SEQ ID NO: 466 - protein, 10 aa, Homo sapiens
WQRMSPSNQT

SEQ ID NO: 467 - protein, 10 aa, Homo sapiens
WERMSPSNQT

SEQ ID NO: 468 - protein, 10 aa, Homo sapiens
WGRMSPSNQT

SEQ ID NO: 469 - protein, 10 aa, Homo sapiens
WHRMSPSNQT

SEQ ID NO: 470 - protein, 10 aa, Homo sapiens
WIRMSPSNQT

SEQ ID NO: 471 - protein, 10 aa, Homo sapiens
WLRMSPSNQT

SEQ ID NO: 472 - protein, 10 aa, Homo sapiens
WKRMSPSNQT

SEQ ID NO: 473 - protein, 10 aa, Homo sapiens
WMRMSPSNQT

SEQ ID NO: 474 - protein, 10 aa, Homo sapiens
WFRMSPSNQT

SEQ ID NO: 475 - protein, 10 aa, Homo sapiens
WPRMSPSNQT

SEQ ID NO: 476 - protein, 10 aa, Homo sapiens
WSRMSPSNQT

SEQ ID NO: 477 - protein, 10 aa, Homo sapiens
WTRMSPSNQT

SEQ ID NO: 478 - protein, 10 aa, Homo sapiens
WWRMSPSNQT

SEQ ID NO: 479 - protein, 10 aa, Homo sapiens
WYRMSPSNQT

SEQ ID NO: 480 - protein, 10 aa, Homo sapiens
WVRMSPSNQT

SEQ ID NO: 481 - protein, 10 aa, Homo sapiens
AYRMSPSNQT

SEQ ID NO: 482 - protein, 10 aa, Homo sapiens
RYRMSPSNQT

SEQ ID NO: 483 - protein, 10 aa, Homo sapiens
NYRMSPSNQT

SEQ ID NO: 484 - protein, 10 aa, Homo sapiens
DYRMSPSNQT

SEQ ID NO: 485 - protein, 10 aa, Homo sapiens
CYRMSPSNQT

SEQ ID NO: 486 - protein, 10 aa, Homo sapiens
QYRMSPSNQT

SEQ ID NO: 487 - protein, 10 aa, Homo sapiens
EYRMSPSNQT

SEQ ID NO: 488 - protein, 10 aa, Homo sapiens
GYRMSPSNQT

SEQ ID NO: 489 - protein, 10 aa, Homo sapiens
HYRMSPSNQT

SEQ ID NO: 490 - protein, 10 aa, Homo sapiens
IYRMSPSNQT

SEQ ID NO: 491 - protein, 10 aa, Homo sapiens
LYRMSPSNQT

SEQ ID NO: 492 - protein, 10 aa, Homo sapiens
KYRMSPSNQT

SEQ ID NO: 493 - protein, 10 aa, Homo sapiens
MYRMSPSNQT

SEQ ID NO: 494 - protein, 10 aa, Homo sapiens
FYRMSPSNQT

SEQ ID NO: 495 - protein, 10 aa, Homo sapiens
PYRMSPSNQT

SEQ ID NO: 496 - protein, 10 aa, Homo sapiens
SYRMSPSNQT

SEQ ID NO: 497 - protein, 10 aa, Homo sapiens
TYRMSPSNQT

SEQ ID NO: 498 - protein, 10 aa, Homo sapiens
WYRMSPSNQT

SEQ ID NO: 499 - protein, 10 aa, Homo sapiens
YYRMSPSNQT

SEQ ID NO: 500 - protein, 10 aa, Homo sapiens
VYRMSPSNQT

SEQ ID NO: 501 - protein, 20 aa, Homo sapiens
METDTLLLWVLLLWVPGSTG

SEQ ID NO: 502 - protein, 20 aa, Homo sapiens
MYRMQLLSCIALSLALVTNS

SEQ ID NO: 503 - protein, 15 aa, Artificial Sequence
  Synthetic sequence
GGGGSGGGGSGGGGS

SEQ ID NO: 504 - protein, 16 aa, Artificial Sequence
  Synthetic sequence
GGGGSLVPRGSGGGGS

SEQ ID NO: 505 - protein, 6 aa, Artificial Sequence
  Synthetic sequence
GSGSGS

SEQ ID NO: 506 - protein, 8 aa, Artificial Sequence
  Synthetic sequence
GSGSGSGS

SEQ ID NO: 507 - protein, 14 aa, Artificial Sequence
  Synthetic sequence
GGGGSLVPRGSGGG

SEQ ID NO: 508 - protein, 10 aa, Artificial Sequence
  Synthetic sequence
GSGGHMGSGG

SEQ ID NO: 509 - protein, 11 aa, Artificial Sequence
  Synthetic sequence
GGSGGSGGSGG

SEQ ID NO: 510 - protein, 5 aa, Artificial Sequence
  Synthetic sequence
GGSGG

SEQ ID NO: 511 - protein, 8 aa, Artificial Sequence
  Synthetic sequence
GGSGGGGG

SEQ ID NO: 512 - protein, 18 aa, Artificial Sequence
  Synthetic sequence
GGGSEGGGSEGGGSEGGG

SEQ ID NO: 513 - protein, 8 aa, Artificial Sequence
  Synthetic sequence
AAGAATAA

SEQ ID NO: 514 - protein, 5 aa, Artificial Sequence
  Synthetic sequence
GGGGG

SEQ ID NO: 515 - protein, 5 aa, Artificial Sequence
  Synthetic sequence
GGSSG

SEQ ID NO: 516 - protein, 11 aa, Artificial Sequence
  Synthetic sequence
GSGGGTGGGSG

SEQ ID NO: 517 - protein, 2 aa, Artificial Sequence
  Synthetic sequence
GT

SEQ ID NO: 518 - protein, 26 aa, Artificial Sequence
  Synthetic sequence
GSGSGSGSGGSGGSGGSGGSGGSGGS

SEQ ID NO: 519 - protein, 14 aa, Artificial Sequence
  Synthetic sequence
GSGGSGSGGSGGSG

SEQ ID NO: 520 - protein, 22 aa, Artificial Sequence
  Synthetic sequence
VKQTLNFDLLKLAGDVESNPGP

SEQ ID NO: 521 - protein, 20 aa, Artificial Sequence
  Synthetic sequence
QCTNYALLKLAGDVESNPGP

SEQ ID NO: 522 - protein, 19 aa, Artificial Sequence
  Synthetic sequence
ATNFSLLKQAGDVEENPGP

SEQ ID NO: 523 - protein, 20 aa, Artificial Sequence
  Synthetic sequence
HYAGYFADLLIHDIETNPGP

SEQ ID NO: 524 - protein, 25 aa, Artificial Sequence
  Synthetic sequence
GIFNAHYAGYFADLLIHDIETNPGP

SEQ ID NO: 525 - protein, 25 aa, Artificial Sequence
  Synthetic sequence
KAVRGYHADYYKQRLIHDVEMNPGP

SEQ ID NO: 526 - protein, 20 aa, Artificial Sequence
  Synthetic sequence
GATNFSLLKLAGDVELNPGP

SEQ ID NO: 527 - protein, 18 aa, Artificial Sequence
  Synthetic sequence
EGRGSLLTCGDVEENPGP

SEQ ID NO: 528 - protein, 19 aa, Artificial Sequence
  Synthetic sequence
AARQMLLLLSGDVETNPGP

SEQ ID NO: 529 - protein, 20 aa, Artificial Sequence
  Synthetic sequence
FLRKRTQLLMSGDVESNPGP

SEQ ID NO: 530 - protein, 20 aa, Artificial Sequence
  Synthetic sequence
GSWTDILLLLSGDVETNPGP

SEQ ID NO: 531 - protein, 19 aa, Artificial Sequence
  Synthetic sequence
TRAEEDELIRAGIESNPGP

SEQ ID NO: 532 - protein, 20 aa, Artificial Sequence
  Synthetic sequence
AKFQIDKILISGDVELNPGP

SEQ ID NO: 533 - protein, 20 aa, Artificial Sequence
  Synthetic sequence
SKFQIDKILISGDIELNPGP

SEQ ID NO: 534 - protein, 20 aa, Artificial Sequence
  Synthetic sequence
SSIIRTKMLVSGDVEENPGP

SEQ ID NO: 535 - protein, 20 aa, Artificial Sequence
  Synthetic sequence
CDAQRQKLLLSGDIEQNPGP

SEQ ID NO: 536 - DNA, 668 bp, Artificial Sequence
  Synthetic sequence
gcgatctgacggttcactaaacgagctctgcttatataggcctcccaccgtacacgccacctcgacatactcgagtagttattaatagtaatcaattacggggtcattagttcatagcccatatatggagttccgcgttacataacttacggtaaatggcccgcctggctgaccgcccaacgacccccgcccattgacgtcaataatgacgtatgttcccatagtaacgccaatagggactttccattgacgtcaatgggtggagtatttacggtaaactgcccacttggcagtacatcaagtgtatcatatgccaagtacgccccctattgacgtcaatgacggtaaatggcccgcctggcattatgcccagtacatgaccttatgggactttcctacttggcagtacatctacgtattagtcatcgctattaccatggtgatgcggttttggcagtacatcaatgggcgtggatagcggtttgactcacggggatttccaagtctccaccccattgacgtcaatgggagtttgttttggcaccaaaatcaacgggactttccaaaatgtcgtaacaactccgccccattgacgcaaatgggcggtaggcgtgtacggtgggaggtctatataagcagagctggtttagtgaaccgtcagatccgct

SEQ ID NO: 537 - protein, 34 aa, Artificial Sequence
  Synthetic sequence
METDTLLLWVLLLWVPGSTGTAHPSPSPRSAGQF

SEQ ID NO: 538 - protein, 59 aa, Artificial Sequence
  Synthetic sequence
METDTLLLWVLLLWVPGSTGEYRMSPSNQTGGGGSGGGGSGGGGSTAHPSPSPRSAGQF

SEQ ID NO: 539 - protein, 59 aa, Artificial Sequence
  Synthetic sequence
METDTLLLWVLLLWVPGSTGYYRMSPSNQTGGGGSGGGGSGGGGSTAHPSPSPRSAGQF

SEQ ID NO: 540 - protein, 34 aa, Artificial Sequence
  Synthetic sequence
METDTLLLWVLLLWVPGSTGTRYPSPSPKPEGRF

SEQ ID NO: 541 - protein, 59 aa, Artificial Sequence
  Synthetic sequence
METDTLLLWVLLLWVPGSTGWNRLSPSNQTGGGGSGGGGSGGGGSTRYPSPSPKPEGRF

SEQ ID NO: 542 - protein, 107 aa, Artificial Sequence
  Synthetic sequence
METDTLLLWVLLLWVPGSTGTAHPSPSPRSAGQFTAHPSPSPRSAGQFTAHPSPSPRSAGQFGGGGSGGGGSGGGGSEYRMSPSNQTEYRMSPSNQTEYRMSPSNQT

SEQ ID NO: 543 - protein, 107 aa, Artificial Sequence
  Synthetic sequence
METDTLLLWVLLLWVPGSTGEYRMSPSNQTEYRMSPSNQTEYRMSPSNQTGGGGSGGGGSGGGGSTAHPSPSPRSAGQFTAHPSPSPRSAGQFTAHPSPSPRSAGQF

SEQ ID NO: 544 - protein, 231 aa, Homo sapiens
ISAMVRSPPCPSCPAPEFLGGPSVFLFPPKPKDTLMISRTPEVTCVVVDVSQEDPEVQFNWYVDGVEVHNAKTKPREEQFNSTYRVVSVLTVLHQDWLNGKEYKCKVSNKGLPSSIEKTISKAKGQPREPQVYTLPPSQEEMTKNQVSLTCLVKGFYPSDIAVEWESNGQPENNYKTTPPVLDSDGSFFLYSRLTVDKSRWQEGNVFSCSVMHEALHNHYTQKSLSLSPGK

SEQ ID NO: 545 - protein, 229 aa, Mus musculus
ISAMVRSGCKPCICTVPEVSSVFIFPPKPKDVLTITLTPKVTCVVVDISKDDPEVQFSWFVDDVEVHTAQTQPREEQFNSTFRSVSELPIMHQDWLNGKEFKCRVNSAAFPAPIEKTISKTKGRPKAPQVYTIPPPKEQMAKDKVSLTCMITDFFPEDITVEWQWNGQPAENYKNTQPIMDTDGSYFVYSKLNVQKSNWEAGNTFTCSVLHEGLHNHHTEKSLSHSPGK

SEQ ID NO: 546 - protein, 265 aa, Artificial Sequence
  Synthetic sequence
MYRMQLLSCIALSLALVTNSTAHPSPSPRSAGQFISAMVRSPPCPSCPAPEFLGGPSVFLFPPKPKDTLMISRTPEVTCVVVDVSQEDPEVQFNWYVDGVEVHNAKTKPREEQFNSTYRVVSVLTVLHQDWLNGKEYKCKVSNKGLPSSIEKTISKAKGQPREPQVYTLPPSQEEMTKNQVSLTCLVKGFYPSDIAVEWESNGQPENNYKTTPPVLDSDGSFFLYSRLTVDKSRWQEGNVFSCSVMHEALHNHYTQKSLSLSPGK

SEQ ID NO: 547 - protein, 290 aa, Artificial Sequence
  Synthetic sequence
MYRMQLLSCIALSLALVTNSEYRMSPSNQTGGGGSGGGGSGGGGSTAHPSPSPRSAGQFISAMVRSPPCPSCPAPEFLGGPSVFLFPPKPKDTLMISRTPEVTCVVVDVSQEDPEVQFNWYVDGVEVHNAKTKPREEQFNSTYRVVSVLTVLHQDWLNGKEYKCKVSNKGLPSSIEKTISKAKGQPREPQVYTLPPSQEEMTKNQVSLTCLVKGFYPSDIAVEWESNGQPENNYKTTPPVLDSDGSFFLYSRLTVDKSRWQEGNVFSCSVMHEALHNHYTQKSLSLSPGK

SEQ ID NO: 548 - protein, 290 aa, Artificial Sequence
  Synthetic sequence
MYRMQLLSCIALSLALVTNSYYRMSPSNQTGGGGSGGGGSGGGGSTAHPSPSPRSAGQFISAMVRSPPCPSCPAPEFLGGPSVFLFPPKPKDTLMISRTPEVTCVVVDVSQEDPEVQFNWYVDGVEVHNAKTKPREEQFNSTYRVVSVLTVLHQDWLNGKEYKCKVSNKGLPSSIEKTISKAKGQPREPQVYTLPPSQEEMTKNQVSLTCLVKGFYPSDIAVEWESNGQPENNYKTTPPVLDSDGSFFLYSRLTVDKSRWQEGNVFSCSVMHEALHNHYTQKSLSLSPGK

SEQ ID NO: 549 - protein, 263 aa, Artificial Sequence
  Synthetic sequence
MYRMQLLSCIALSLALVTNSTRYPSPSPKPEGRFISAMVRSGCKPCICTVPEVSSVFIFPPKPKDVLTITLTPKVTCVVVDISKDDPEVQFSWFVDDVEVHTAQTQPREEQFNSTFRSVSELPIMHQDWLNGKEFKCRVNSAAFPAPIEKTISKTKGRPKAPQVYTIPPPKEQMAKDKVSLTCMITDFFPEDITVEWQWNGQPAENYKNTQPIMDTDGSYFVYSKLNVQKSNWEAGNTFTCSVLHEGLHNHHTEKSLSHSPGK

SEQ ID NO: 550 - protein, 288 aa, Artificial Sequence
  Synthetic sequence
MYRMQLLSCIALSLALVTNSWNRLSPSNQTGGGGSGGGGSGGGGSTRYPSPSPKPEGRFISAMVRSGCKPCICTVPEVSSVFIFPPKPKDVLTITLTPKVTCVVVDISKDDPEVQFSWFVDDVEVHTAQTQPREEQFNSTFRSVSELPIMHQDWLNGKEFKCRVNSAAFPAPIEKTISKTKGRPKAPQVYTIPPPKEQMAKDKVSLTCMITDFFPEDITVEWQWNGQPAENYKNTQPIMDTDGSYFVYSKLNVQKSNWEAGNTFTCSVLHEGLHNHHTEKSLSHSPGK

SEQ ID NO: 551 - DNA, 1335 bp, Homo sapiens
gagtaattcatacaaaaggactcgcccctgccttggggaatcccagggaccgtcgttaaactcccactaacgtagaacccagagatcgctgcgttcccgccccctcacccgcccgctctcgtcatcactgaggtggagaagagcatgcgtgaggctccggtgcccgtcagtgggcagagcgcacatcgcccacagtccccgagaagttggggggaggggtcggcaattgaaccggtgcctagagaaggtggcgcggggtaaactgggaaagtgatgtcgtgtactggctccgcctttttcccgagggtgggggagaaccgtatataagtgcagtagtcgccgtgaacgttctttttcgcaacgggtttgccgccagaacacaggtaagtgccgtgtgtggttcccgcgggcctggcctctttacgggttatggcccttgcgtgccttgaattacttccacgcccctggctgcagtacgtgattcttgatcccgagcttcgggttggaagtgggtgggagagttcgaggccttgcgcttaaggagccccttcgcctcgtgcttgagttgaggcctggcttgggcgctggggccgccgcgtgcgaatctggtggcaccttcgcgcctgtctcgctgctttcgataagtctctagccatttaaaatttttgatgacctgctgcgacgctttttttctggcaagatagtcttgtaaatgcgggccaagatctgcacactggtatttcggtttttggggccgcgggcggcgacggggcccgtgcgtcccagcgcacatgttcggcgaggcggggcctgcgagcgcggccaccgagaatcggacgggggtagtctcaagctggccggcctgctctggtgcctggcctcgcgccgccgtgtatcgccccgccctgggcggcaaggctggcccggtcggcaccagttgcgtgagcggaaagatggccgcttcccggccctgctgcagggagctcaaaatggaggacgcggcgctcgggagagcgggcgggtgagtcacccacacaaaggaaaagggcctttccgtcctcagccgtcgcttcatgtgactccacggagtaccgggcgccgtccaggcacctcgattagttctcgagcttttggagtacgtcgtctttaggttggggggaggggttttatgcgatggagtttccccacactgagtgggtggagactgaagttaggccagcttggcacttgatgtaattctccttggaatttgccctttttgagtttggatcttggttcattctcaagcctcagacagtggttcaaagtttttttcttccatttcaggtgtcgtga

SEQ ID NO: 552 - DNA, 601 bp, Artificial Sequence
  Synthetic sequence
cctctcccccccccccctctccctcccccccccctaacgttactggccgaagccgcttggaataaggccggtgtgcgtttgtctatatgttattttccaccatattgccgtcttttggcaatgtgagggcccggaaacctggccctgtcttcttgacgagcattcctaggggtctttcccctctcgccaaaggaatgcaaggtctgttgaatgtcgtgaaggaagcagttcctctggaagcttcttgaagacaaacaacgtctgtagcgaccctttgcaggcagcggaaccccccacctggcgacaggtgcctctgcggccaaaagccacgtgtataagatacacctgcaaaggcggcacaaccccagtgccacgttgtgagttggatagttgtggaaagagtcaaatggctctcctcaagcgtattcaacaaggggctgaaggatgcccagaaggtaccccattgtatgggatctgatctggggcctcggtgcacatgctttacatgtgtttagtcgaggttaaaaaaacgtctaggccccccgaaccacggggacgtggttttcctttgaaaaacacgatgataagcttgccacaaccc

SEQ ID NO: 553 - DNA, 536 bp, Human cytomegalovirus
ccgcgttacataacttacggtaaatggcccgcctggctgaccgcccaacgacccccgcccattgacgtcaataatgacgtatgttcccatagtaacgccaatagggactttccattgacgtcaatgggtggagtatttacggtaaactgcccacttggcagtacatcaagtgtatcatatgccaagtacgccccctattgacgtcaatgacggtaaatggcccgcctggcattatgcccagtacatgaccttatgggactttcctacttggcagtacatctacgtattagtcatcgctattaccatggtgatgcggttttggcagtacatcaatgggcgtggatagcggtttgactcacggggatttccaagtctccaccccattgacgtcaatgggagtttgttttggcaccaaaatcaacgggactttccaaaatgtcgtaacaactccgccccattgacgcaaatgggcggtaggcgtgtacggtgggaggtctatataagcagagctggtttagtgaaccgtcagatccgct

SEQ ID NO: 554 - protein, 22 aa, Artificial Sequence
  Synthetic sequence
GSGATNFSLLKQAGDVEENPGP

SEQ ID NO: 555 - DNA, 1433 bp, Artificial Sequence
  Synthetic sequence
atgtcgggcgtcgggggagagggagttccctctgcgcttgcgattctagcctcgtggggctggacgttcgacacgccaaaccacgagtcggggatatcgccagatacgactcccgcagattccattcggggtgccgctgtggcctcacctgaccaacctttacacgggggcccggaacgggaggccacagcgccgtctttctccccaacgcgcgcggatgacggcccgccctgtaccgacgggccctacgtgacgtttgataccctgtttatggtgtcgtcgatcgacgaattagggcgtcgccagctcacggacaccatccgcaaggacctgcggttgtcgctggccaagtttagcattgcgtgcaccaagacctcctcgttttcgggaaacgccccgcgccaccacagacgcggggcgttccagcgcggcacgcgggcgccgcgcagcaacaaaagcctccagatgtttgtgttgtgcaaacgcgcccacgccgctcgagtgcgagagcagcttcgggtcgttattcagtcccgcaagccgcgcaagtattacacgcgatcttcggacgggcggctctgccccgccgtccccgtgttcgtccacgagttcgtctcgtccgagccaatgcgcctccaccgagataacgtcatgctggcctcgggggccgagtaaccgccccccccccatgccaccctcactgcccgtcgcgcgtgtttgatgttaataaataacacataaatttggctggttgtttgttgtctttaatggaccgcccgcaagggggggggggcatttcagtgtcgggtgacgagcgcgatccggccgggatcctaggaccccaaaagtttgtctgcgtattccagggcggggctcagttgaatctcccgcagcacctctaccagcaggtccgcggtgggctggagaaactcggccgtcccggggcaggcggttgtcgggggtggaggcgcggcgcccaccccgtgtgccgcgcctggcgtctcctctgggggcgacccgtaaatggttgcagtgatgtaaatggtgtccgcggtccagaccacggtcaaaatgccggccgtggcgctccgggcgctttcgccgcgcgaggagctgacccaggagtcgaacggatacgcgtacatatgggcgtcccacccgcgttcgagcttctggttgctgtcccggcctataaagcggtaggcacaaaattcggcgcgacagtcgataatcaccaacagcccaatgggggtgtgctggataacaacgcctccgcgcggcaggcggtcctggcgctcccggccccgtaccatgatcgcgcgggtgccgtactcaaaaacatgcaccacctgcgcggcgtcgggcagtgcgctggtcagcgaggccctggcgtggcataggctatacgcgatggtcgtctgtggattggacat

SEQ ID NO: 556 - DNA, 1533 bp, Artificial Sequence
  Synthetic sequence
ggccctcaatccctaatacatttcagtgatggggtagtccagtgagccacatttgttgccttgttcagcacgcactctgtcagggagctggtgccggccttccgcttgaagccagagttgcagatgtatctctcccgggaatacaggctgtaagacttcacccagatgtctgcgtgctccacgctcattggaggtgggcaggtgatgccccttgtagcggggggtctcagcagcagcagcagcagcagggcaggcagtcccagggtccgacatcctctagcgcggcgtggagccatggtggcgaattctccaggcgatctgacggttcactaaacgagctctgcttatataggcctcccaccgtacacgccacctcgacatactcgagtagttattaatagtaatcaattacggggtcattagttcatagcccatatatggagttccgcgttacataacttacggtaaatggcccgcctggctgaccgcccaacgacccccgcccattgacgtcaataatgacgtatgttcccatagtaacgccaatagggactttccattgacgtcaatgggtggagtatttacggtaaactgcccacttggcagtacatcaagtgtatcatatgccaagtacgccccctattgacgtcaatgacggtaaatggcccgcctggcattatgcccagtacatgaccttatgggactttcctacttggcagtacatctacgtattagtcatcgctattaccatggtgatgcggttttggcagtacatcaatgggcgtggatagcggtttgactcacggggatttccaagtctccaccccattgacgtcaatgggagtttgttttggcaccaaaatcaacgggactttccaaaatgtcgtaacaactccgccccattgacgcaaatgggcggtaggcgtgtacggtgggaggtctatataagcagagctggtttagtgaaccgtcagatccgctagggatcctctagtcagctgacgcgtgctagcgcggccgcatcgataagcttgccaccatgcggatttccaagccccatctgcgctccatttccatccagtgttacctgtgcctgctgctgaatagccattttctgaccgaagccggcatccacgtgttcatcctgggctgcttttccgccggcctgccaaagaccgaggcaaactgggtgaatgtgatctctgacctgaagaagatcgaggatctgatccagagcatgcacatcgacgccaccctgtacacagagtccgatgtgcacccttcttgcaaggtgacagccatgaagtgtttcctgctggagctgcaggtcatctctctggagagcggcgacgcctctatccacgataccgtggagaacctgatcatcctggccaacaatagcctgagctccaacggcaatgtgacagagtccggctgcaaggagtgtgaggagctggaggagaagaatatcaaagagttcctgcagagtttcgtccatatcgtccagatgtttatcaatacttcctaagtcga

SEQ ID NO: 557 - DNA, 2304 bp, Artificial Sequence
  Synthetic sequence
ggcccttacagatggtgactacagttttccaggtcctcgtctcttgatgaagttccccaggtgacgggcagggcctccatggcctccatctccacagaggccagagggggggtctgtctggacttcagataacaggccagcagggacacggcgctcaggccgcacagcagcactgtagaggtggagatggccactgtggtgtcggagtggccctgtgggtacacgcctggaggctggtggctggcagatgctgtcagctcccaattcttggctgtggtctgagaaggggtgccgtggctagactcgtgggagctgatctctgtggtgcctgtggatgggctcttagaaggcatcagctgggagccaggcacgattgctgctgtggttgctgcggtattgttagaggatgggctagatgctgcaggctccttgccggatgggctcagagactctggctgtggtgtcacgccggctgtggtcacggtgctgggtggtgcgggccgctggtgcaccagggcgggatcccggatgcacttcagagagggtgtggtccagtgggccacattggtggccttgttcagcacgcactctgtcagggagctggtgccggccttcctcttaaagccgctgttgcagatgtatctctcccgagaatacagggagtagctcttcacccagatgtcggcgtgctccacggacatagggggtggacatgtgatgcctgcctgctgtctgctggtccggtggtggtgacactgggggcaattctccattgtcctcagcctcacgcatgcctcgtgggtctgcacctcgtggttgaaagactcggagattctgctccggcctgccagcacggccaggcgatcccttgcgtcgcgtgttgcagggggcctcagcagcagcagtaataacagggcgggcaggcccagggtgcgacagcccctggctctccttggtgccattgctgctgctccgcaggacacggcgggtgagccgggtcttgcgctgcccagtccgggtggtggaggggatctctgttcggggacctgtcttcctgccagtctcatggtggcgaattctccaggcgatctgacggttcactaaacgagctctgcttatataggcctcccaccgtacacgccacctcgacatactcgagtagttattaatagtaatcaattacggggtcattagttcatagcccatatatggagttccgcgttacataacttacggtaaatggcccgcctggctgaccgcccaacgacccccgcccattgacgtcaataatgacgtatgttcccatagtaacgccaatagggactttccattgacgtcaatgggtggagtatttacggtaaactgcccacttggcagtacatcaagtgtatcatatgccaagtacgccccctattgacgtcaatgacggtaaatggcccgcctggcattatgcccagtacatgaccttatgggactttcctacttggcagtacatctacgtattagtcatcgctattaccatggtgatgcggttttggcagtacatcaatgggcgtggatagcggtttgactcacggggatttccaagtctccaccccattgacgtcaatgggagtttgttttggcaccaaaatcaacgggactttccaaaatgtcgtaacaactccgccccattgacgcaaatgggcggtaggcgtgtacggtgggaggtctatataagcagagctggtttagtgaaccgtcagatccgctagggatcctctagtcagctgacgcgtgctagcgcggccgcatcgataagcttgccaccatgcggatttccaagccccatctgcgctccatttccatccagtgttacctgtgcctgctgctgaatagccattttctgaccgaagccggcatccacgtgttcatcctgggctgcttttccgccggcctgccaaagaccgaggcaaactgggtgaatgtgatctctgacctgaagaagatcgaggatctgatccagagcatgcacatcgacgccaccctgtacacagagtccgatgtgcacccttcttgcaaggtgacagccatgaagtgtttcctgctggagctgcaggtcatctctctggagagcggcgacgcctctatccacgataccgtggagaacctgatcatcctggccaacaatagcctgagctccaacggcaatgtgacagagtccggctgcaaggagtgtgaggagctggaggagaagaatatcaaagagttcctgcagagtttcgtccatatcgtccagatgtttatcaatacttcctaagtcga

SEQ ID NO: 558 - DNA, 1842 bp, Artificial Sequence
  Synthetic sequence
ggcccttatttttccagtgcggacacctctttttccagggctgacacctccttttccagggctgagacttctttttccagggcagacacctccttctccagggcagacacctcggagccgccgccgccggatcctcctcctccgcttcctcctcctccatcccggatacacttcagggagggtgtggtccagtgggccacatttgtggccttgttcagcacgcactctgtcagggagctggtgccggccttcctcttgaagccgctgttgcagatgtatctctcccgagaatacaggctgtaagacttcacccagatgtctgcgtgctccacgctcattggaggtgggcaggtgatgccccttgtagcaggtggtctcagcagcagcagcagcagcagggcaggcagtcccagtgtgcgacatcctcgggctcttctaggggccatggtggcgaattctccaggcgatctgacggttcactaaacgagctctgcttatataggcctcccaccgtacacgccacctcgacatactcgagtagttattaatagtaatcaattacggggtcattagttcatagcccatatatggagttccgcgttacataacttacggtaaatggcccgcctggctgaccgcccaacgacccccgcccattgacgtcaataatgacgtatgttcccatagtaacgccaatagggactttccattgacgtcaatgggtggagtatttacggtaaactgcccacttggcagtacatcaagtgtatcatatgccaagtacgccccctattgacgtcaatgacggtaaatggcccgcctggcattatgcccagtacatgaccttatgggactttcctacttggcagtacatctacgtattagtcatcgctattaccatggtgatgcggttttggcagtacatcaatgggcgtggatagcggtttgactcacggggatttccaagtctccaccccattgacgtcaatgggagtttgttttggcaccaaaatcaacgggactttccaaaatgtcgtaacaactccgccccattgacgcaaatgggcggtaggcgtgtacggtgggaggtctatataagcagagctggtttagtgaaccgtcagatccgctagggatcctctagtcagctgacgcgtgctagcgcggccgcatcgataagcttgccaccatgcggatttccaaacctcacctgcgatctatctccatccagtgctatctgtgcctgctgctgaactctcatttcctgaccgaagccggcatccacgtgttcatcctgggctgctttagcgccggcctgccaaagaccgaggcaaactgggtgaatgtgatctctgacctgaagaagatcgaggatctgatccagagcatgcacatcgacgccaccctgtacacagagtccgatgtgcacccttcttgcaaggtgacagccatgaagtgtttcctgctggagctgcaggtcatctctctggagagcggcgacgcctccatccacgataccgtggagaacctgatcatcctggccaacaatagcctgagctccaacggcaatgtgacagagtccggctgcaaggagtgtgaggagctggaggagaagaacatcaaggagttcctgcagtcttttgtgcacatcgtgcagatgtttatcaataccagcggaggaggaggatccggcggaggaggctctggcggcggcggcagctgtggcggcaaggtgtccgccctgaaggagaaggtgtctgccctgaaggaaaaagtgtccgctctgaaggaaaaggtgtccgcactgaaagaaaaggtctccgccctgaaggaataagtcga

SEQ ID NO: 559 - DNA, 2613 bp, Artificial Sequence
  Synthetic sequence
ggcccttatttttccagtgcggacacctctttttccagtgctgacacctccttctccagggctgacacttctttttccagggcgctcacctctttttccagggcagacacctcggagccgccgccgccggagcctcctcctccgcttcctcctcctcccaggtggtgggaacaattctccagatcctcgtcgcgagaggatgtgccccaggtcactggcagggcctccattgcctccatctccacagatgccagaggtggggtctgcctggacttcagataacaggccagcaggctcacggcagacaggccgcacagcagcactgtggaggtgctgatggccactgtggtgtcggagtggccctgtgggtacacgcctggaggctggtgagaggcggatgctgtcagctcccagttcttggctgtggtctgagaaggggtgccgtggctagactcgtgggagctgatctctgtggtgccggtgcttggagacttggaaggcatcagctgggagccaggcacgattgctgctgtggttgctgcggtattgttagaggatgggctagatgctgcaggctccttgccgcttggagacagggactctggctgtggtgtcactcctgctgtggtcacggtgctgggtggtgcgggccgctggtgcaccagggcgggatcccggatgcacttcagagagggtgtggtccagtgggccacattggtggccttgttcagcacgcactctgtcagggagctggtgccggccttccgcttaaagccgctgttgcagatgtatctctcccgagaatacaggctgtaagacttcacccagatgtcggcgtgctccacggacatagggggtggacatgtgatgcctgcctgctgtctgctggtccggtggtggtgacactgggggcaattctccattgtcctcagcctcacgcatgcctcgtgggtctgcacctcgtggttgaaggactcgctgattctgctccggcctgccagcacggccaggcgatcccttgcgtcgcgtgttgcagggggcctcagcagcagcagtaataacagggcgggcaggcccagggtgcgacagcccctggctctccttggtgccattgctgctgctccgcaggacacagcgggactgccgggtcttgcactgcccagcccaggaggaggaggggatctctgctcggggacctgccttccagccagccgcatggtggcgaattctccaggcgatctgacggttcactaaacgagctctgcttatataggcctcccaccgtacacgccacctcgacatactcgagtagttattaatagtaatcaattacggggtcattagttcatagcccatatatggagttccgcgttacataacttacggtaaatggcccgcctggctgaccgcccaacgacccccgcccattgacgtcaataatgacgtatgttcccatagtaacgccaatagggactttccattgacgtcaatgggtggagtatttacggtaaactgcccacttggcagtacatcaagtgtatcatatgccaagtacgccccctattgacgtcaatgacggtaaatggcccgcctggcattatgcccagtacatgaccttatgggactttcctacttggcagtacatctacgtattagtcatcgctattaccatggtgatgcggttttggcagtacatcaatgggcgtggatagcggtttgactcacggggatttccaagtctccaccccattgacgtcaatgggagtttgttttggcaccaaaatcaacgggactttccaaaatgtcgtaacaactccgccccattgacgcaaatgggcggtaggcgtgtacggtgggaggtctatataagcagagctggtttagtgaaccgtcagatccgctagggatcctctagtcagctgacgcgtgctagcgcggccgcatcgataagcttgccaccatgcggatttccaaacctcacctgcgatctatctccatccagtgctatctgtgcctgctgctgaactctcatttcctgaccgaagccggcatccacgtgttcatcctgggctgctttagcgccggcctgccaaagaccgaggcaaactgggtgaatgtgatctctgacctgaagaagatcgaggatctgatccagagcatgcacatcgacgccaccctgtacacagagtccgatgtgcacccttcttgcaaggtgacagccatgaagtgtttcctgctggagctgcaggtcatctctctggagagcggcgacgcctccatccacgataccgtggagaacctgatcatcctggccaacaatagcctgagctccaacggcaatgtgacagagtccggctgcaaggagtgtgaggagctggaggagaagaacatcaaggagttcctgcagtcttttgtgcacatcgtgcagatgtttatcaataccagcggaggaggaggatccggcggaggaggctctggcggcggcggcagctgtggcggcaaggtgtccgccctgaaggagaaggtgtctgccctgaaggaaaaagtgtccgctctgaaggaaaaggtgtccgcactgaaagaaaaggtctccgccctgaaggaataagtcga

SEQ ID NO: 560 - DNA, 3135 bp, Artificial Sequence
  Synthetic sequence
gagtaattcatacaaaaggactcgcccctgccttggggaatcccagggaccgtcgttaaactcccactaacgtagaacccagagatcgctgcgttcccgccccctcacccgcccgctctcgtcatcactgaggtggagaagagcatgcgtgaggctccggtgcccgtcagtgggcagagcgcacatcgcccacagtccccgagaagttggggggaggggtcggcaattgaaccggtgcctagagaaggtggcgcggggtaaactgggaaagtgatgtcgtgtactggctccgcctttttcccgagggtgggggagaaccgtatataagtgcagtagtcgccgtgaacgttctttttcgcaacgggtttgccgccagaacacaggtaagtgccgtgtgtggttcccgcgggcctggcctctttacgggttatggcccttgcgtgccttgaattacttccacgcccctggctgcagtacgtgattcttgatcccgagcttcgggttggaagtgggtgggagagttcgaggccttgcgcttaaggagccccttcgcctcgtgcttgagttgaggcctggcttgggcgctggggccgccgcgtgcgaatctggtggcaccttcgcgcctgtctcgctgctttcgataagtctctagccatttaaaatttttgatgacctgctgcgacgctttttttctggcaagatagtcttgtaaatgcgggccaagatctgcacactggtatttcggtttttggggccgcgggcggcgacggggcccgtgcgtcccagcgcacatgttcggcgaggcggggcctgcgagcgcggccaccgagaatcggacgggggtagtctcaagctggccggcctgctctggtgcctggcctcgcgccgccgtgtatcgccccgccctgggcggcaaggctggcccggtcggcaccagttgcgtgagcggaaagatggccgcttcccggccctgctgcagggagctcaaaatggaggacgcggcgctcgggagagcgggcgggtgagtcacccacacaaaggaaaagggcctttccgtcctcagccgtcgcttcatgtgactccacggagtaccgggcgccgtccaggcacctcgattagttctcgagcttttggagtacgtcgtctttaggttggggggaggggttttatgcgatggagtttccccacactgagtgggtggagactgaagttaggccagcttggcacttgatgtaattctccttggaatttgccctttttgagtttggatcttggttcattctcaagcctcagacagtggttcaaagtttttttcttccatttcaggtgtcgtgaactagaagctttattgcggtagtttatcacagttaaattgctaacgcagtcagtgcttctgacacaacagtctcgaacttaagctgcagtgactctcttaaggtagccttgcagaagttggtcgtgaggcactgggcaggtaagtatcaaggttacaagacaggtttaaggagaccaatagaaactgggcttgtcgagacagagaagactcttgcgtttctgataggcacctattggtcttactgacatccactttgcctttctctccacaggtgtccactcccagttcaattacagctcttaaggctagagtacttaatacgactcactataggctagcgccaccatgcggatttccaagccccatctgcgctccatttccatccagtgttacctgtgcctgctgctgaatagccattttctgaccgaagccggcatccacgtgttcatcctgggctgcttttccgccggcctgccaaagaccgaggcaaactgggtgaatgtgatctctgacctgaagaagatcgaggatctgatccagagcatgcacatcgacgccaccctgtacacagagtccgatgtgcacccttcttgcaaggtgacagccatgaagtgtttcctgctggagctgcaggtcatctctctggagagcggcgacgcctctatccacgataccgtggagaacctgatcatcctggccaacaatagcctgagctccaacggcaatgtgacagagtccggctgcaaggagtgtgaggagctggaggagaagaatatcaaagagttcctgcagagtttcgtccatatcgtccagatgtttatcaatacttcctaagaattcacgcgtcgagcatgcatctagggcggccaattccgcccctctcccccccccccctctccctcccccccccctaacgttactggccgaagccgcttggaataaggccggtgtgcgtttgtctatatgttattttccaccatattgccgtcttttggcaatgtgagggcccggaaacctggccctgtcttcttgacgagcattcctaggggtctttcccctctcgccaaaggaatgcaaggtctgttgaatgtcgtgaaggaagcagttcctctggaagcttcttgaagacaaacaacgtctgtagcgaccctttgcaggcagcggaaccccccacctggcgacaggtgcctctgcggccaaaagccacgtgtataagatacacctgcaaaggcggcacaaccccagtgccacgttgtgagttggatagttgtggaaagagtcaaatggctctcctcaagcgtattcaacaaggggctgaaggatgcccagaaggtaccccattgtatgggatctgatctggggcctcggtgcacatgctttacatgtgtttagtcgaggttaaaaaaacgtctaggccccccgaaccacggggacgtggttttcctttgaaaaacacgatgataagcttgccacaacccgggatcctctagagtcgacgccaccatggctccacgccgcgctagaggatgtcggaccctgggactgcctgccctgctgctgctgctgctgctgagaccccccgctacaaggggcatcacctgcccacctccaatgagcgtggagcacgcagacatctgggtgaagtcttacagcctgtattcccgggagagatacatctgcaactctggcttcaagcggaaggccggcaccagctccctgacagagtgcgtgctgaacaaggcaacaaatgtggctcactggactaccccatcactgaaatgtattagggattgagtcga

SEQ ID NO: 561 - DNA, 3906 bp, Artificial Sequence
  Synthetic sequence
gagtaattcatacaaaaggactcgcccctgccttggggaatcccagggaccgtcgttaaactcccactaacgtagaacccagagatcgctgcgttcccgccccctcacccgcccgctctcgtcatcactgaggtggagaagagcatgcgtgaggctccggtgcccgtcagtgggcagagcgcacatcgcccacagtccccgagaagttggggggaggggtcggcaattgaaccggtgcctagagaaggtggcgcggggtaaactgggaaagtgatgtcgtgtactggctccgcctttttcccgagggtgggggagaaccgtatataagtgcagtagtcgccgtgaacgttctttttcgcaacgggtttgccgccagaacacaggtaagtgccgtgtgtggttcccgcgggcctggcctctttacgggttatggcccttgcgtgccttgaattacttccacgcccctggctgcagtacgtgattcttgatcccgagcttcgggttggaagtgggtgggagagttcgaggccttgcgcttaaggagccccttcgcctcgtgcttgagttgaggcctggcttgggcgctggggccgccgcgtgcgaatctggtggcaccttcgcgcctgtctcgctgctttcgataagtctctagccatttaaaatttttgatgacctgctgcgacgctttttttctggcaagatagtcttgtaaatgcgggccaagatctgcacactggtatttcggtttttggggccgcgggcggcgacggggcccgtgcgtcccagcgcacatgttcggcgaggcggggcctgcgagcgcggccaccgagaatcggacgggggtagtctcaagctggccggcctgctctggtgcctggcctcgcgccgccgtgtatcgccccgccctgggcggcaaggctggcccggtcggcaccagttgcgtgagcggaaagatggccgcttcccggccctgctgcagggagctcaaaatggaggacgcggcgctcgggagagcgggcgggtgagtcacccacacaaaggaaaagggcctttccgtcctcagccgtcgcttcatgtgactccacggagtaccgggcgccgtccaggcacctcgattagttctcgagcttttggagtacgtcgtctttaggttggggggaggggttttatgcgatggagtttccccacactgagtgggtggagactgaagttaggccagcttggcacttgatgtaattctccttggaatttgccctttttgagtttggatcttggttcattctcaagcctcagacagtggttcaaagtttttttcttccatttcaggtgtcgtgaactagaagctttattgcggtagtttatcacagttaaattgctaacgcagtcagtgcttctgacacaacagtctcgaacttaagctgcagtgactctcttaaggtagccttgcagaagttggtcgtgaggcactgggcaggtaagtatcaaggttacaagacaggtttaaggagaccaatagaaactgggcttgtcgagacagagaagactcttgcgtttctgataggcacctattggtcttactgacatccactttgcctttctctccacaggtgtccactcccagttcaattacagctcttaaggctagagtacttaatacgactcactataggctagcgccaccatgcggatttccaagccccatctgcgctccatttccatccagtgttacctgtgcctgctgctgaatagccattttctgaccgaagccggcatccacgtgttcatcctgggctgcttttccgccggcctgccaaagaccgaggcaaactgggtgaatgtgatctctgacctgaagaagatcgaggatctgatccagagcatgcacatcgacgccaccctgtacacagagtccgatgtgcacccttcttgcaaggtgacagccatgaagtgtttcctgctggagctgcaggtcatctctctggagagcggcgacgcctctatccacgataccgtggagaacctgatcatcctggccaacaatagcctgagctccaacggcaatgtgacagagtccggctgcaaggagtgtgaggagctggaggagaagaatatcaaagagttcctgcagagtttcgtccatatcgtccagatgtttatcaatacttcctaagaattcacgcgtcgagcatgcatctagggcggccaattccgcccctctcccccccccccctctccctcccccccccctaacgttactggccgaagccgcttggaataaggccggtgtgcgtttgtctatatgttattttccaccatattgccgtcttttggcaatgtgagggcccggaaacctggccctgtcttcttgacgagcattcctaggggtctttcccctctcgccaaaggaatgcaaggtctgttgaatgtcgtgaaggaagcagttcctctggaagcttcttgaagacaaacaacgtctgtagcgaccctttgcaggcagcggaaccccccacctggcgacaggtgcctctgcggccaaaagccacgtgtataagatacacctgcaaaggcggcacaaccccagtgccacgttgtgagttggatagttgtggaaagagtcaaatggctctcctcaagcgtattcaacaaggggctgaaggatgcccagaaggtaccccattgtatgggatctgatctggggcctcggtgcacatgctttacatgtgtttagtcgaggttaaaaaaacgtctaggccccccgaaccacggggacgtggttttcctttgaaaaacacgatgataagcttgccacaacccgggatcctctagagtcgacgccaccatgagactggcaggaagacaggtccccgaacagagatcccctccaccacccggactgggcagcgcaagacccggctcacccgccgtgtcctgcggagcagcagcaatggcaccaaggagagccaggggctgtcgcaccctgggcctgcccgccctgttattactgctgctgctgaggccccctgcaacacgcgacgcaagggatcgcctggccgtgctggcaggccggagcagaatctccgagtctttcaaccacgaggtgcagacccacgaggcatgcgtgaggctgaggacaatggagaattgcccccagtgtcaccaccaccggaccagcagacagcaggcaggcatcacatgtccaccccctatgtccgtggagcacgccgacatctgggtgaagagctactccctgtattctcgggagagatacatctgcaacagcggctttaagaggaaggccggcaccagctccctgacagagtgcgtgctgaacaaggccaccaatgtggcccactggaccacaccctctctgaagtgcatccgggatcccgccctggtgcaccagcggcccgcaccacccagcaccgtgaccacagccggcgtgacaccacagccagagtctctgagcccatccggcaaggagcctgcagcatctagcccatcctctaacaataccgcagcaaccacagcagcaatcgtgcctggctcccagctgatgccttctaagagcccatccacaggcaccacagagatcagctcccacgagtctagccacggcaccccttctcagaccacagccaagaattgggagctgacagcatctgccagccaccagcctccaggcgtgtacccacagggccactccgacaccacagtggccatctccacctctacagtgctgctgtgcggcctgagcgccgtgtccctgctggcctgttatctgaagtccagacagaccccccctctggcctctgtggagatggaggccatggaggccctgcccgtcacctggggaacttcatcaagagacgaggacctggaaaactgtagtcaccatctgtaagtcga

SEQ ID NO: 562 - DNA, 3487 bp, Artificial Sequence
  Synthetic sequence
gagtaattcatacaaaaggactcgcccctgccttggggaatcccagggaccgtcgttaaactcccactaacgtagaacccagagatcgctgcgttcccgccccctcacccgcccgctctcgtcatcactgaggtggagaagagcatgcgtgaggctccggtgcccgtcagtgggcagagcgcacatcgcccacagtccccgagaagttggggggaggggtcggcaattgaaccggtgcctagagaaggtggcgcggggtaaactgggaaagtgatgtcgtgtactggctccgcctttttcccgagggtgggggagaaccgtatataagtgcagtagtcgccgtgaacgttctttttcgcaacgggtttgccgccagaacacaggtaagtgccgtgtgtggttcccgcgggcctggcctctttacgggttatggcccttgcgtgccttgaattacttccacgcccctggctgcagtacgtgattcttgatcccgagcttcgggttggaagtgggtgggagagttcgaggccttgcgcttaaggagccccttcgcctcgtgcttgagttgaggcctggcttgggcgctggggccgccgcgtgcgaatctggtggcaccttcgcgcctgtctcgctgctttcgataagtctctagccatttaaaatttttgatgacctgctgcgacgctttttttctggcaagatagtcttgtaaatgcgggccaagatctgcacactggtatttcggtttttggggccgcgggcggcgacggggcccgtgcgtcccagcgcacatgttcggcgaggcggggcctgcgagcgcggccaccgagaatcggacgggggtagtctcaagctggccggcctgctctggtgcctggcctcgcgccgccgtgtatcgccccgccctgggcggcaaggctggcccggtcggcaccagttgcgtgagcggaaagatggccgcttcccggccctgctgcagggagctcaaaatggaggacgcggcgctcgggagagcgggcgggtgagtcacccacacaaaggaaaagggcctttccgtcctcagccgtcgcttcatgtgactccacggagtaccgggcgccgtccaggcacctcgattagttctcgagcttttggagtacgtcgtctttaggttggggggaggggttttatgcgatggagtttccccacactgagtgggtggagactgaagttaggccagcttggcacttgatgtaattctccttggaatttgccctttttgagtttggatcttggttcattctcaagcctcagacagtggttcaaagtttttttcttccatttcaggtgtcgtgaactagaagctttattgcggtagtttatcacagttaaattgctaacgcagtcagtgcttctgacacaacagtctcgaacttaagctgcagtgactctcttaaggtagccttgcagaagttggtcgtgaggcactgggcaggtaagtatcaaggttacaagacaggtttaaggagaccaatagaaactgggcttgtcgagacagagaagactcttgcgtttctgataggcacctattggtcttactgacatccactttgcctttctctccacaggtgtccactcccagttcaattacagctcttaaggctagagtacttaatacgactcactataggctagcgccaccatgcggatttccaaacctcacctgcgatctatctccatccagtgctatctgtgcctgctgctgaactctcatttcctgaccgaagccggcatccacgtgttcatcctgggctgctttagcgccggcctgccaaagaccgaggcaaactgggtgaatgtgatctctgacctgaagaagatcgaggatctgatccagagcatgcacatcgacgccaccctgtacacagagtccgatgtgcacccttcttgcaaggtgacagccatgaagtgtttcctgctggagctgcaggtcatctctctggagagcggcgacgcctccatccacgataccgtggagaacctgatcatcctggccaacaatagcctgagctccaacggcaatgtgacagagtccggctgcaaggagtgtgaggagctggaggagaagaacatcaaggagttcctgcagtcttttgtgcacatcgtgcagatgtttatcaataccagcggaggaggaggatccggcggaggaggctctggcggcggcggcagctgtggcggcaaggtgtccgccctgaaggagaaggtgtctgccctgaaggaaaaagtgtccgctctgaaggaaaaggtgtccgcactgaaagaaaaggtctccgccctgaaggaataagaattcacgcgtcgagcatgcatctagggcggccaattccgcccctctcccccccccccctctccctcccccccccctaacgttactggccgaagccgcttggaataaggccggtgtgcgtttgtctatatgttattttccaccatattgccgtcttttggcaatgtgagggcccggaaacctggccctgtcttcttgacgagcattcctaggggtctttcccctctcgccaaaggaatgcaaggtctgttgaatgtcgtgaaggaagcagttcctctggaagcttcttgaagacaaacaacgtctgtagcgaccctttgcaggcagcggaaccccccacctggcgacaggtgcctctgcggccaaaagccacgtgtataagatacacctgcaaaggcggcacaaccccagtgccacgttgtgagttggatagttgtggaaagagtcaaatggctctcctcaagcgtattcaacaaggggctgaaggatgcccagaaggtaccccattgtatgggatctgatctggggcctcggtgcacatgctttacatgtgtttagtcgaggttaaaaaaacgtctaggccccccgaaccacggggacgtggttttcctttgaaaaacacgatgataagcttgccacaacccgggatcctctagagtcgacgccaccatggcccctagaagagcccgaggatgtcgcacactgggactgcctgccctgctgctgctgctgctgctgagaccacctgctacaaggggcatcacctgcccacctccaatgagcgtggagcacgcagacatctgggtgaagtcttacagcctgtattctcgggagagatacatctgcaacagcggcttcaagaggaaggccggcaccagctccctgacagagtgcgtgctgaacaaggccacaaatgtggcccactggaccacaccctccctgaagtgtatccgggatggaggaggaggaagcggaggaggaggatccggcggcggcggctccgaggtgtctgccctggagaaggaggtgtctgccctggaaaaagaagtctcagccctggaaaaggaggtgtcagccctggaaaaagaggtgtccgcactggaaaaataagtcgaagtcgggacctttttctccacaggcgtgacctttttattcagc

SEQ ID NO: 563 - DNA, 4215 bp, Artificial Sequence
  Synthetic sequence
gagtaattcatacaaaaggactcgcccctgccttggggaatcccagggaccgtcgttaaactcccactaacgtagaacccagagatcgctgcgttcccgccccctcacccgcccgctctcgtcatcactgaggtggagaagagcatgcgtgaggctccggtgcccgtcagtgggcagagcgcacatcgcccacagtccccgagaagttggggggaggggtcggcaattgaaccggtgcctagagaaggtggcgcggggtaaactgggaaagtgatgtcgtgtactggctccgcctttttcccgagggtgggggagaaccgtatataagtgcagtagtcgccgtgaacgttctttttcgcaacgggtttgccgccagaacacaggtaagtgccgtgtgtggttcccgcgggcctggcctctttacgggttatggcccttgcgtgccttgaattacttccacgcccctggctgcagtacgtgattcttgatcccgagcttcgggttggaagtgggtgggagagttcgaggccttgcgcttaaggagccccttcgcctcgtgcttgagttgaggcctggcttgggcgctggggccgccgcgtgcgaatctggtggcaccttcgcgcctgtctcgctgctttcgataagtctctagccatttaaaatttttgatgacctgctgcgacgctttttttctggcaagatagtcttgtaaatgcgggccaagatctgcacactggtatttcggtttttggggccgcgggcggcgacggggcccgtgcgtcccagcgcacatgttcggcgaggcggggcctgcgagcgcggccaccgagaatcggacgggggtagtctcaagctggccggcctgctctggtgcctggcctcgcgccgccgtgtatcgccccgccctgggcggcaaggctggcccggtcggcaccagttgcgtgagcggaaagatggccgcttcccggccctgctgcagggagctcaaaatggaggacgcggcgctcgggagagcgggcgggtgagtcacccacacaaaggaaaagggcctttccgtcctcagccgtcgcttcatgtgactccacggagtaccgggcgccgtccaggcacctcgattagttctcgagcttttggagtacgtcgtctttaggttggggggaggggttttatgcgatggagtttccccacactgagtgggtggagactgaagttaggccagcttggcacttgatgtaattctccttggaatttgccctttttgagtttggatcttggttcattctcaagcctcagacagtggttcaaagtttttttcttccatttcaggtgtcgtgaactagaagctttattgcggtagtttatcacagttaaattgctaacgcagtcagtgcttctgacacaacagtctcgaacttaagctgcagtgactctcttaaggtagccttgcagaagttggtcgtgaggcactgggcaggtaagtatcaaggttacaagacaggtttaaggagaccaatagaaactgggcttgtcgagacagagaagactcttgcgtttctgataggcacctattggtcttactgacatccactttgcctttctctccacaggtgtccactcccagttcaattacagctcttaaggctagagtacttaatacgactcactataggctagcgccaccatgcggatttccaaacctcacctgcgatctatctccatccagtgctatctgtgcctgctgctgaactctcatttcctgaccgaagccggcatccacgtgttcatcctgggctgctttagcgccggcctgccaaagaccgaggcaaactgggtgaatgtgatctctgacctgaagaagatcgaggatctgatccagagcatgcacatcgacgccaccctgtacacagagtccgatgtgcacccttcttgcaaggtgacagccatgaagtgtttcctgctggagctgcaggtcatctctctggagagcggcgacgcctccatccacgataccgtggagaacctgatcatcctggccaacaatagcctgagctccaacggcaatgtgacagagtccggctgcaaggagtgtgaggagctggaggagaagaacatcaaggagttcctgcagtcttttgtgcacatcgtgcagatgtttatcaataccagcggaggaggaggatccggcggaggaggctctggcggcggcggcagctgtggcggcaaggtgtccgccctgaaggagaaggtgtctgccctgaaggaaaaagtgtccgctctgaaggaaaaggtgtccgcactgaaagaaaaggtctccgccctgaaggaataagaattcacgcgtcgagcatgcatctagggcggccaattccgcccctctcccccccccccctctccctcccccccccctaacgttactggccgaagccgcttggaataaggccggtgtgcgtttgtctatatgttattttccaccatattgccgtcttttggcaatgtgagggcccggaaacctggccctgtcttcttgacgagcattcctaggggtctttcccctctcgccaaaggaatgcaaggtctgttgaatgtcgtgaaggaagcagttcctctggaagcttcttgaagacaaacaacgtctgtagcgaccctttgcaggcagcggaaccccccacctggcgacaggtgcctctgcggccaaaagccacgtgtataagatacacctgcaaaggcggcacaaccccagtgccacgttgtgagttggatagttgtggaaagagtcaaatggctctcctcaagcgtattcaacaaggggctgaaggatgcccagaaggtaccccattgtatgggatctgatctggggcctcggtgcacatgctttacatgtgtttagtcgaggttaaaaaaacgtctaggccccccgaaccacggggacgtggttttcctttgaaaaacacgatgataagcttgccacaacccgggatcctctagagtcgacgccaccatgcggctggctggaaggcaggtccccgagcagagatcccctcctcctcctgggctgggcagtgcaagacccggcagtcccgctgtgtcctgcggagcagcagcaatggcaccaaggagagccaggggctgtcgcaccctgggcctgcccgccctgttattactgctgctgctgaggccccctgcaacacgcgacgcaagggatcgcctggccgtgctggcaggccggagcagaatcagcgagtccttcaaccacgaggtgcagacccacgaggcatgcgtgaggctgaggacaatggagaattgcccccagtgtcaccaccaccggaccagcagacagcaggcaggcatcacatgtccaccccctatgtccgtggagcacgccgacatctgggtgaagtcttacagcctgtattctcgggagagatacatctgcaacagcggctttaagcggaaggccggcaccagctccctgacagagtgcgtgctgaacaaggccaccaatgtggcccactggaccacaccctctctgaagtgcatccgggatcccgccctggtgcaccagcggcccgcaccacccagcaccgtgaccacagcaggagtgacaccacagccagagtccctgtctccaagcggcaaggagcctgcagcatctagcccatcctctaacaataccgcagcaaccacagcagcaatcgtgcctggctcccagctgatgccttccaagtctccaagcaccggcaccacagagatcagctcccacgagtctagccacggcaccccttctcagaccacagccaagaactgggagctgacagcatccgcctctcaccagcctccaggcgtgtacccacagggccactccgacaccacagtggccatcagcacctccacagtgctgctgtgcggcctgtctgccgtgagcctgctggcctgttatctgaagtccaggcagaccccacctctggcatctgtggagatggaggcaatggaggccctgccagtgacctggggcacatcctctcgcgacgaggatctggagaattgttcccaccacctgggaggaggaggaagcggaggaggaggctccggcggcggcggctccgaggtgtctgccctggaaaaagaggtgagcgccctggaaaaagaagtgtcagccctggagaaggaggtgtcagcactggaaaaagaggtgtccgcactggaaaaataagtcga

SEQ ID NO: 564 - DNA, 3425 bp, Artificial Sequence
  Synthetic sequence
acattgattattgactagttattaatagtaatcaattacggggtcattagttcatagcccatatatggagttccgcgttacataacttacggtaaatggcccgcctggctgaccgcccaacgacccccgcccattgacgtcaataatgacgtatgttcccatagtaacgccaatagggactttccattgacgtcaatgggtggagtatttacggtaaactgcccacttggcagtacatcaagtgtatcatatgccaagtacgccccctattgacgtcaatgacggtaaatggcccgcctggcattatgcccagtacatgaccttatgggactttcctacttggcagtacatctacgtattagtcatcgctattaccatggtgatgcggttttggcagtacatcaatgggcgtggatagcggtttgactcacggggatttccaagtctccaccccattgacgtcaatgggagtttgttttggcaccaaaatcaacgggactttccaaaatgtcgtaacaactccgccccattgacgcaaatgggcggtaggcgtgtacggtgggaggtctatataagcagagctctctggctaactagagaacccactgcttactggcttatcgaaattaatacgactcactatagggagacccaagctggctagcgtttaaacttaagcttggtaccgagctcggatccactagtccagtgtggtggaattcgccaccatgtgccctcagaaactgactatctcatggttcgcaatcgtgctgctggtctcacccctgatggctatgtgggaactggaaaaggatgtgtacgtggtggaggtggactggacacccgatgcccctggcgagacagtgaacctgacatgcgacacccccgaggaggacgacatcacctggacatccgatcagcggcacggcgtgatcggctctggcaagaccctgacaatcaccgtgaaggagttcctggacgccggccagtacacatgtcacaagggcggcgagacactgagccactcccacctgctgctgcacaagaaggagaacggcatctggtccacagagatcctgaagaacttcaagaataagacctttctgaagtgcgaggcccccaattattctggccggttcacctgtagctggctggtgcagagaaacatggacctgaagtttaatatcaagagctcctctagctcccctgatagcagggcagtgacatgcggaatggcatctctgagcgccgagaaggtgaccctggaccagagagattacgagaagtattccgtgtcttgccaggaggatgtgacatgtcccaccgccgaggagacactgcctatcgagctggccctggaggcaaggcagcagaacaagtacgagaattatagcacctccttctttatcagagacatcatcaagccagatccccctaagaacctgcagatgaagcccctgaagaacagccaggtcgaggtgagctgggagtaccctgactcttggagcacaccacactcttatttcagcctgaagttctttgtgaggatccagcgcaagaaggagaagatgaaggagacagaggagggctgcaaccagaagggcgcctttctggtggagaagacatccaccgaggtgcagtgcaagggaggaaacgtgtgcgtgcaggcacaggatagatactataattctagctgctctaagtgggcctgcgtgccctgtagggtgcgctccggaggcggcggctctggaggaggaggaagcggaggaggaggaagcatgtgccagtccaggtacctgctgttcctggccaccctggccctgctgaaccacctgtccctggcacgcgtgatcccagtgtctggaccagcccggtgcctgtcccagtctagaaatctgctgaagaccacagacgatatggtgaagacagccagggagaagctgaagcactattcctgtaccgccgaggacatcgatcacgaggacatcacacgcgatcagacatccaccctgaagacctgcctgcctctggagctgcacaagaacgagtcttgtctggccacacgggagacaagctctaccacaagaggcagctgcctgccaccccagaagacatccctgatgatgaccctgtgcctgggcagcatctacgaggacctgaagatgtatcagacagagtttcaggccatcaatgccgccctgcagaaccacaatcaccagcagatcatcctggacaagggcatgctggtggccatcgatgagctgatgcagtccctgaaccacaatggcgagacactgaggcagaagcctccagtgggcgaggccgatccttaccgcgtgaagatgaagctgtgcatcctgctgcacgccttcagcacaagggtggtgaccatcaaccgcgtgatgggctatctgagctccgccggaggaggaggatccggcggaggaggctctggcggcggcggcagcggctccggcgccaccaacttttctctgctgaagcaggcaggcgacgtggaggagaatccaggacccatgaggatcagcaagccacacctgcgctctatcagcatccagtgctacctgtgcctgctgctgaatagccacttcctgacagaggccggcatccacgtgttcatcctgggctgtttttccgccggcctgccaaagaccgaggccaactgggtgaatgtgatctctgacctgaagaagatcgaggatctgatccagagcatgcacatcgacgccacactgtataccgagagcgatgtgcacccctcctgcaaggtgaccgccatgaagtgttttctgctggagctgcaggtcatcagcctggagtctggcgacgccagcatccacgatacagtggagaacctgatcatcctggccaacaatagcctgtctagcaacggcaatgtgaccgagtccggctgcaaggagtgtgaggagctggaggagaagaacatcaaggagttcctgcagtcctttgtgcacatcgtgcagatgttcatcaatacatccggcggcggcggctccggcggcggagggagcggaggaggcggctccggctctggcgccaccaactttagcctgctgaagcaggccggcgacgtggaagaaaatcctggaccaatggcacctaggagagcaaggggatgcagaaccctgggcctgccagccctgttattactgctgctgctgaggccccctgcaacaaggggaatcacctgtccaccccctatgagcgtggagcacgccgacatctgggtgaagagctactccctgtattctcgggagagatacatctgcaatagcggcttcaagcggaaggccggcacatcctctctgaccgagtgcgtgctgaacaaagcaacaaacgtggctcattggacaacaccatccctgaagtgcatccgcgactaagat

SEQ ID NO: 565 - DNA, 3912 bp, Artificial Sequence
  Synthetic sequence
acattgattattgactagttattaatagtaatcaattacggggtcattagttcatagcccatatatggagttccccgcctggctgaccgcccaacgacccccgcccattgacgtcaataatgacgtatgttcccatagtaacgccaatagggactttccattgacgtcaatgggtggagtatttacggtaaactgcccacttggcagtacatcaagtgtatcatatgccaagtacgccccctattgacgtcaatgacggtaaatggcccgcctggcattatgcccagtacatgaccttatgggactttcctacttggcagtacatctacgtattagtcatcgctattaccatggtgatgcggttttggcagtacatcaatgggcgtggatagcggtttgactcacggggatttccaagtctccaccccattgacgtcaatgggagtttgttttggcaccaaaatcaacgggactttccaaaatgtcgtaacaactccgccccattgacgcaaatgggcggtaggcgtgtacggtgggaggtctatataagcagagctctctggctaactagagaacccactgcttactggcttatcgaaattaatacgactcactatagggagacccaagctggctagcgtttaaacttaagcttggtaccgagctcggatccactagtccagtgtggtggaattcgccaccatgtgccctcagaagctgactatctcttggtttgctattgtgctgctggtctcacccctgatggctatgtgggaactggaaaaggatgtgtacgtggtggaggtggactggacaccagatgcccccggcgagacagtgaacctgacatgcgacacccccgaggaggacgacatcacctggacatctgatcagaggcacggcgtgatcggaagcggcaagaccctgacaatcaccgtgaaggagttcctggacgccggccagtacacatgtcacaagggcggcgagacactgtctcacagccacctgctgctgcacaagaaggagaacggcatctggagcacagagatcctgaagaacttcaagaataagacctttctgaagtgcgaggccccaaattattccggcaggttcacctgttcttggctggtgcagcgcaacatggacctgaagtttaatatcaagagctcctctagctcccccgattccagggcagtgacatgcggaatggcatccctgtctgccgagaaggtgaccctggaccagcgcgattacgagaagtatagcgtgtcctgccaggaggatgtgacatgtcctaccgccgaggagacactgccaatcgagctggccctggaggccaggcagcagaacaagtacgagaattattctaccagcttctttatccgcgacatcatcaagccagatccccctaagaacctgcagatgaagcccctgaagaacagccaggtcgaggtgtcttgggagtacccagactcctggtctacaccccactcttatttcagcctgaagttctttgtgaggatccagcgcaagaaggagaagatgaaggagacagaggagggctgcaaccagaagggcgcctttctggtggagaagacatccaccgaggtgcagtgcaagggaggaaacgtgtgcgtgcaggcacaggatagatactataattctagctgcagcaagtgggcctgcgtgccttgtagggtgcgcagcggaggaggaggatccggaggaggcggctctggaggaggaggatctatgtgccagagccggtacctgctgttcctggccaccctggccctgctgaaccacctgagcctggcaagagtgatccccgtgagcggaccagcaaggtgcctgagccagtccagaaatctgctgaagaccacagacgatatggtgaagacagcccgggagaagctgaagcactatagctgtaccgccgaggacatcgatcacgaggacatcacaagagatcagacatctaccctgaagacctgcctgcccctggagctgcacaagaacgagagctgtctggccacacgggagacaagctctaccacaagaggctcttgcctgccaccccagaagacaagcctgatgatgaccctgtgcctgggcagcatctacgaggacctgaagatgtatcagaccgagtttcaggccatcaatgccgccctgcagaaccacaatcaccagcagatcatcctggacaagggcatgctggtggccatcgatgagctgatgcagagcctgaaccacaatggcgagacactgaggcagaagcctccagtgggagaggcagatccatacagagtgaagatgaagctgtgcatcctgctgcacgccttctccacaagggtggtgaccatcaaccgcgtgatgggctatctgagctccgccggaggaggaggaagcggcggaggaggcagcggcggcggcggctctggcagcggcgccaccaactttagcctgctgaagcaggcaggcgacgtggaggagaatccaggacccatgaggatctccaagccccacctgcgctccatctctatccagtgctacctgtgcctgctgctgaacagccacttcctgacagaggccggcatccacgtgttcatcctgggctgtttttctgccggcctgcctaagaccgaggccaactgggtgaatgtgatcagcgacctgaagaagatcgaggatctgatccagtccatgcacatcgacgccacactgtataccgagtctgatgtgcacccaagctgcaaggtgaccgccatgaagtgttttctgctggagctgcaggtcatcagcctggagtctggcgacgccagcatccacgatacagtggagaacctgatcatcctggccaacaattccctgtctagcaacggcaatgtgaccgagtctggctgcaaggagtgtgaggagctggaggagaagaacatcaaggagttcctgcagagctttgtgcacatcgtgcagatgttcatcaatacaagcggaggcggaggatctggcggcggcggcagtggcggaggaggaagcggctccggcgccaccaacttttccctgctgaagcaggccggcgacgtggaagaaaatcctggaccaatggcacctaggagagcaaggggatgcagaaccctgggcctgccagccctgttattactgctgctgctgaggccccctgcaacaaggggaatcacctgtccaccccctatgagcgtggagcacgccgacatctgggtgaagtcttacagcctgtattcccgggagagatacatctgcaactctggcttcaagaggaaggccggcacatcctctctgaccgagtgcgtgctgaacaaggccaccaatgtggcccactggaccacaccctctctgaagtgcatccgggaccccgccctggtgcaccagcggcccgcaccacccagcacagtgaccacagcaggagtgaccccacagcctgagtccctgtctccaagcggcaaggagccagcagcaagctccccttctagcaacaatacagcagcaaccacagcagcaatcgtgcctggctcccagctgatgccctccaagtctcctagcaccggcaccacagagatctcctctcacgagagctcccacggcacacccagccagaccacagccaagaattgggagctgaccgcatccgcctctcaccagcctccaggcgtgtaccctcagggccactccgataccacagtggccatcagcacatccaccgtgctgctgtgcggcctgagcgccgtgtccctgctggcctgttatctgaagagcaggcagaccccacctctggcatccgtggagatggaggccatggaggccctgcccgtcacctgggggacatcatcacgggacgaagacctggagaactgctcacatcatctgtaagat

SEQ ID NO: 566 - DNA, 3808 bp, Artificial Sequence
  Synthetic sequence
acattgattattgactagttattaatagtaatcaattacggggtcattagttcatagcccatatatggagttccgcgttacataacttacggtaaatggctgtaactaataactgatcaataattatcattagttaatgccccagtaatcaagtatcgggtatatacctcaaggccgcctggctgaccgcccaacgacccccgcccattgacgtcaataatgacgtatgttcccatagtaacgccaatagggactttccattgacgtcaatgggtggagtatttacggtaaactgcccacttggcagtacatcaagtgtatcatatgccaagtacgccccctattgacgtcaatgacggtaaatggcccgcctggcattatgcccagtacatgaccttatgggactttcctacttggcagtacatctacgtattagtcatcgctattaccatggtgatgcggttttggcagtacatcaatgggcgtggatagcggtttgactcacggggatttccaagtctccaccccattgacgtcaatgggagtttgttttggcaccaaaatcaacgggactttccaaaatgtcgtaacaactccgccccattgacgcaaatgggcggtaggcgtgtacggtgggaggtctatataagcagagctctctggctaactagagaacccactgcttactggcttatcgaaattaatacgactcactatagggagacccaagctggctagcgtttaaacttaagcttggtaccgagctcggatccactagtccagtgtggtggaattcgccaccatgtgccctcagaaactgacaatctcctggttcgctatcgtcctgctggtctctcctctgatggctatgtgggaactggaaaaagatgtgtacgtggtggaggtggactggacacccgatgcccctggcgagacagtgaacctgacatgcgacacccccgaggaggacgacatcacctggacatccgatcagaggcacggcgtgatcggctctggcaagaccctgacaatcaccgtgaaggagttcctggacgccggccagtacacatgtcacaagggcggcgagacactgagccactcccacctgctgctgcacaagaaggagaacggcatctggtccacagagatcctgaagaacttcaagaataagacctttctgaagtgcgaggcccccaattatagcggccggttcacctgttcctggctggtgcagagaaacatggacctgaagtttaatatcaagagctcctctagctcccctgatagcagggcagtgacatgcggaatggcatctctgagcgccgagaaggtgaccctggaccagagagattacgagaagtattccgtgtcttgccaggaggatgtgacatgtcccaccgccgaggagacactgcctatcgagctggccctggaggcaaggcagcagaacaagtacgagaattatagcacctccttctttatcagagacatcatcaagccagatccccctaagaacctgcagatgaagcccctgaagaacagccaggtcgaggtgtcttgggagtaccctgactcttggagcacaccacactcttatttcagcctgaagttctttgtgaggatccagcgcaagaaggagaagatgaaggagacagaggagggctgtaaccagaagggcgcctttctggtggagaagacatccaccgaggtgcagtgcaagggaggaaacgtgtgcgtgcaggcacaggatcggtactataattctagctgctctaagtgggcctgcgtgccctgtagggtgcgcagcggaggaggaggatccggaggaggcggctctggaggaggaggatctatgtgccagagcaggtacctgctgttcctggccaccctggccctgctgaaccacctgtccctggcacgcgtgatcccagtgtctggaccagcccggtgcctgtcccagtctagaaatctgctgaagaccacagacgatatggtgaagacagccagggagaagctgaagcactatagctgtaccgccgaggacatcgatcacgaggacatcacacgcgatcagacatccaccctgaagacctgcctgcctctggagctgcacaagaacgagtcttgtctggccacacgggagacaagctctaccacaagaggcagctgcctgccaccccagaagacatccctgatgatgaccctgtgcctgggcagcatctacgaggacctgaagatgtatcagacagagtttcaggccatcaatgccgccctgcagaaccacaatcaccagcagatcatcctggacaagggcatgctggtggccatcgatgagctgatgcagtccctgaaccacaatggcgagacactgaggcagaagcctccagtgggcgaggccgatccttaccgcgtgaagatgaagctgtgcatcctgctgcacgccttcagcacaagggtggtgaccatcaaccgcgtgatgggctatctgagctccgccggaggaggaggaagcggcggaggaggcagcggcggcggcggcagcggctccggcgccaccaacttttctctgctgaagcaggcaggcgacgtggaggagaatccaggacccatgaggatcagcaagccacacctgcgctctatcagcatccagtgctacctgtgcctgctgctgaatagccacttcctgacagaggccggcatccacgtgttcatcctgggctgtttttccgccggcctgccaaagaccgaggccaactgggtgaatgtgatctctgacctgaagaagatcgaggatctgatccagagcatgcacatcgacgccacactgtataccgagtctgatgtgcaccccagctgcaaggtgaccgccatgaagtgttttctgctggagctgcaggtcatcagcctggagtctggcgacgcctccatccacgatacagtggagaacctgatcatcctggccaacaatagcctgtctagcaacggcaatgtgaccgagtccggctgcaaggagtgtgaggagctggaggagaagaacatcaaggagttcctgcagagctttgtgcacatcgtgcagatgttcatcaatacctccggcggcggaggatctggcggcggcggctccggcgggggaggatcctgcggcggcaaggtgtctgccctgaaggagaaggtgagcgccctgaaggaaaaggtgtccgccctgaaggagaaggtgtctgccctgaaggaaaaggtgagcgccctgaaggagggcggcggaggatctgggggcggcggctccgggggaggaggatccggctctggcgccacaaacttctccctgctgaagcaggccggcgacgtggaagaaaatcctggaccaatggcacctaggagagcaaggggatgcagaaccctgggcctgccagccctgttattactgctgctgctgaggccccctgcaacaaggggaatcacctgtccaccccctatgagcgtggagcacgccgacatctgggtgaagagctactccctgtattctcgggagagatacatctgcaatagcggctttaagcggaaggccggcacatcctctctgaccgagtgcgtgctgaacaaggccaccaatgtggcccactggaccacaccctccctgaagtgcatcagagatggcggcggcggatccggaggaggcgggtctggcggcggcggcagcgaggtgtccgccctggagaaggaggtgagcgccctggaaaaagaggtgagtgctctggaaaaggaagtgtctgccctggaaaaggaagtgtctgccctggaaaaatgagat

SEQ ID NO: 567 - DNA, 4247 bp, Artificial Sequence
  Synthetic sequence
acattgattattgactagttattaatagtaatcaattacggggtcattagttcatagcccatatatggagttccgcgttacataacttacggtaaatggcccgcctggctgaccgcccaacgacccccgcccattgacgtcaataatgacgtatgttcccatagtaacgccaatagggactttccattgacgtcaatgggtggagtatttacggtaaactgcccacttggcagtacatcaagtgtatcatatgccaagtacgccccctattgacgtcaatgacggtaaatggcccgcctggcattatgcccagtacatgaccttatgggactttcctacttggcagtacatctacgtattagtcatcgctattaccatggtgatgcggttttggcagtacatcaatgggcgtggatagcggtttgactcacggggatttccaagtctccaccccattgacgtcaatgggagtttgttttggcaccaaaatcaacgggactttccaaaatgtcgtaacaactccgccccattgacgcaaatgggcggtaggcgtgtacggtgggaggtctatataagcagagctctctggctaactagagaacccactgcttactggcttatcgaaattaatacgactcactatagggagacccaagctggctagcgtttaaacttaagcttggtaccgagctcggatccactagtccagtgtggtggaattcgccaccatgtgcccccagaaactgacaatctcttggttcgcaatcgtgctgctggtctcacccctgatggctatgtgggagctggaaaaggatgtgtacgtggtggaggtggactggacaccagatgcccccggcgagacagtgaacctgacatgcgacacccccgaggaggacgacatcacctggacatccgatcagcggcacggcgtgatcggctctggcaagaccctgacaatcaccgtgaaggagttcctggacgccggccagtacacatgtcacaagggcggcgagacactgtcccactctcacctgctgctgcacaagaaggagaacggcatctggagcacagagatcctgaagaacttcaagaataagacctttctgaagtgcgaggccccaaattattccggcaggttcacctgttcttggctggtgcagcgcaacatggacctgaagtttaatatcaagagctcctctagctcccccgattccagggcagtgacatgcggaatggcaagcctgtccgccgagaaggtgaccctggaccagagggattacgagaagtattctgtgagctgccaggaggatgtgacatgtcctaccgccgaggagacactgccaatcgagctggccctggaggccaggcagcagaacaagtacgagaattattccacctctttctttatccgcgacatcatcaagccagatccccctaagaacctgcagatgaagcccctgaagaacagccaggtcgaggtgagctgggagtacccagacagctggtccacaccccactcctatttctctctgaagttctttgtgaggatccagcgcaagaaggagaagatgaaggagacagaggagggctgtaaccagaagggcgcctttctggtggagaagacatccaccgaggtgcagtgcaagggaggaaacgtgtgcgtgcaggcacaggatagatactataattctagctgcagcaagtgggcctgcgtgccttgtagggtgcgctccggaggcggcggctctggaggaggaggaagcggaggaggaggaagcatgtgccagtcccggtacctgctgttcctggccaccctggccctgctgaaccacctgtctctggccagagtgatccctgtgagcggaccagcaaggtgcctgtctcagagcagaaatctgctgaagaccacagacgatatggtgaagacagcccgggagaagctgaagcactatagctgtaccgccgaggacatcgatcacgaggacatcacaagagatcagacatccaccctgaagacctgcctgcccctggagctgcacaagaacgagtcttgtctggccacacgggagacaagctctaccacaagaggctcctgcctgccaccccagaagacatctctgatgatgaccctgtgcctgggcagcatctacgaggacctgaagatgtatcagaccgagtttcaggccatcaatgccgccctgcagaaccacaatcaccagcagatcatcctggacaagggcatgctggtggccatcgatgagctgatgcagagcctgaaccacaatggcgagacactgaggcagaagcctccagtgggagaggcagatccatacagagtgaagatgaagctgtgcatcctgctgcacgccttctccacaagggtggtgaccatcaaccgcgtgatgggctatctgagctccgccggaggaggaggatccggcggaggaggctctggcggcggcggctccggctctggcgccaccaacttttctctgctgaagcaggcaggcgacgtggaggagaatccaggacccatgaggatcagcaagccccacctgcgcagcatctccatccagtgctacctgtgcctgctgctgaatagccacttcctgacagaggccggcatccacgtgttcatcctgggctgtttttccgccggcctgcctaagaccgaggccaactgggtgaatgtgatctctgacctgaagaagatcgaggatctgatccagagcatgcacatcgacgccacactgtataccgagagcgatgtgcacccatcctgcaaggtgaccgccatgaagtgttttctgctggagctgcaggtcatcagcctggagtccggcgacgcaagcatccacgatacagtggagaacctgatcatcctggccaacaatagcctgtctagcaacggcaatgtgaccgagtccggctgcaaggagtgtgaggagctggaggagaagaacatcaaggagttcctgcagtcctttgtgcacatcgtgcagatgttcatcaatacttccggcggcggcggcagtggcggaggaggaagcggaggcggcggctcttgcggcggcaaggtgagcgccctgaaggagaaggtgtccgccctgaaggaaaaggtgtctgccctgaaggagaaggtgagcgccctgaaggaaaaggtgtccgccctgaaggaggggggcggcggcagcggcggaggagggagcgggggaggcggctctggcagcggcgccacaaacttcagcctgctgaagcaggccggcgacgtggaagaaaatcctggaccaatggcacctaggagagcaaggggatgcagaaccctgggcctgccagccctgttattactgctgctgctgaggccccctgcaacaaggggaatcacctgtccaccccctatgagcgtggagcacgccgacatctgggtgaagtcctactctctgtatagccgggagagatacatctgcaattccggctttaagaggaaggccggcacatcctctctgaccgagtgcgtgctgaacaaggccaccaatgtggcccactggaccacaccatccctgaagtgcatccgggaccccgccctggtgcaccagcggcccgcaccaccatctacagtgaccacagcaggagtgaccccacagcctgagagcctgtccccatctggcaaggagccagcagcaagctccccttctagcaacaatacagcagcaaccacagcagcaatcgtgcctggctcccagctgatgcccagcaagtccccttctaccggcaccacagagatctcctctcacgagagctcccacggcacacccagccagaccacagccaagaactgggagctgaccgcaagcgcctcccaccagcctccaggcgtgtaccctcagggccactccgataccacagtggccatctctacaagcaccgtgctgctgtgcggcctgtctgccgtgagcctgctggcctgttatctgaagtctaggcagaccccacctctggcaagcgtggagatggaggcaatggaggccctgccagtgacatggggcacctctagccgcgacgaggatctggagaattgcagccaccacctgggaggaggaggatcaggcggcggcgggtccggcggcggcggatccgaggtgtctgccctggagaaggaggtgtccgccctggaaaaagaagtgtcagccctggagaaagaagtgtcagccctggaaaaagaggtgtctgccctggaaaaataagat

SEQ ID NO: 568 - protein, 897 aa, Artificial Sequence
  Synthetic sequence
MCPQKLTISWFAIVLLVSPLMAMWELEKDVYVVEVDWTPDAPGETVNLTCDTPEEDDITWTSDQRHGVIGSGKTLTITVKEFLDAGQYTCHKGGETLSHSHLLLHKKENGIWSTEILKNFKNKTFLKCEAPNYSGRFTCSWLVQRNMDLKFNIKSSSSSPDSRAVTCGMASLSAEKVTLDQRDYEKYSVSCQEDVTCPTAEETLPIELALEARQQNKYENYSTSFFIRDIIKPDPPKNLQMKPLKNSQVEVSWEYPDSWSTPHSYFSLKFFVRIQRKKEKMKETEEGCNQKGAFLVEKTSTEVQCKGGNVCVQAQDRYYNSSCSKWACVPCRVRSGGGGSGGGGSGGGGSMCQSRYLLFLATLALLNHLSLARVIPVSGPARCLSQSRNLLKTTDDMVKTAREKLKHYSCTAEDIDHEDITRDQTSTLKTCLPLELHKNESCLATRETSSTTRGSCLPPQKTSLMMTLCLGSIYEDLKMYQTEFQAINAALQNHNHQQIILDKGMLVAIDELMQSLNHNGETLRQKPPVGEADPYRVKMKLCILLHAFSTRVVTINRVMGYLSSAGGGGSGGGGSGGGGSGSGATNFSLLKQAGDVEENPGPMRISKPHLRSISIQCYLCLLLNSHFLTEAGIHVFILGCFSAGLPKTEANWVNVISDLKKIEDLIQSMHIDATLYTESDVHPSCKVTAMKCFLLELQVISLESGDASIHDTVENLIILANNSLSSNGNVTESGCKECEELEEKNIKEFLQSFVHIVQMFINTSGGGGSGGGGSGGGGSGSGATNFSLLKQAGDVEENPGPMAPRRARGCRTLGLPALLLLLLLRPPATRGITCPPPMSVEHADIWVKSYSLYSRERYICNSGFKRKAGTSSLTECVLNKATNVAHWTTPSLKCIRD

SEQ ID NO: 569 - protein, 1068 aa, Artificial Sequence
  Synthetic sequence
MCPQKLTISWFAIVLLVSPLMAMWELEKDVYVVEVDWTPDAPGETVNLTCDTPEEDDITWTSDQRHGVIGSGKTLTITVKEFLDAGQYTCHKGGETLSHSHLLLHKKENGIWSTEILKNFKNKTFLKCEAPNYSGRFTCSWLVQRNMDLKFNIKSSSSSPDSRAVTCGMASLSAEKVTLDQRDYEKYSVSCQEDVTCPTAEETLPIELALEARQQNKYENYSTSFFIRDIIKPDPPKNLQMKPLKNSQVEVSWEYPDSWSTPHSYFSLKFFVRIQRKKEKMKETEEGCNQKGAFLVEKTSTEVQCKGGNVCVQAQDRYYNSSCSKWACVPCRVRSGGGGSGGGGSGGGGSMCQSRYLLFLATLALLNHLSLARVIPVSGPARCLSQSRNLLKTTDDMVKTAREKLKHYSCTAEDIDHEDITRDQTSTLKTCLPLELHKNESCLATRETSSTTRGSCLPPQKTSLMMTLCLGSIYEDLKMYQTEFQAINAALQNHNHQQIILDKGMLVAIDELMQSLNHNGETLRQKPPVGEADPYRVKMKLCILLHAFSTRVVTINRVMGYLSSAGGGGSGGGGSGGGGSGSGATNFSLLKQAGDVEENPGPMRISKPHLRSISIQCYLCLLLNSHFLTEAGIHVFILGCFSAGLPKTEANWVNVISDLKKIEDLIQSMHIDATLYTESDVHPSCKVTAMKCFLLELQVISLESGDASIHDTVENLIILANNSLSSNGNVTESGCKECEELEEKNIKEFLQSFVHIVQMFINTSGGGGSGGGGSGGGGSGSGATNFSLLKQAGDVEENPGPMAPRRARGCRTLGLPALLLLLLLRPPATRGITCPPPMSVEHADIWVKSYSLYSRERYICNSGFKRKAGTSSLTECVLNKATNVAHWTTPSLKCIRDPALVHQRPAPPSTVTTAGVTPQPESLSPSGKEPAASSPSSNNTAATTAAIVPGSQLMPSKSPSTGTTEISSHESSHGTPSQTTAKNWELTASASHQPPGVYPQGHSDTTVAISTSTVLLCGLSAVSLLACYLKSRQTPPLASVEMEAMEALPVTWGTSSRDEDLENCSHHL

SEQ ID NO: 570 - protein, 1000 aa, Artificial Sequence
  Synthetic sequence
MCPQKLTISWFAIVLLVSPLMAMWELEKDVYVVEVDWTPDAPGETVNLTCDTPEEDDITWTSDQRHGVIGSGKTLTITVKEFLDAGQYTCHKGGETLSHSHLLLHKKENGIWSTEILKNFKNKTFLKCEAPNYSGRFTCSWLVQRNMDLKFNIKSSSSSPDSRAVTCGMASLSAEKVTLDQRDYEKYSVSCQEDVTCPTAEETLPIELALEARQQNKYENYSTSFFIRDIIKPDPPKNLQMKPLKNSQVEVSWEYPDSWSTPHSYFSLKFFVRIQRKKEKMKETEEGCNQKGAFLVEKTSTEVQCKGGNVCVQAQDRYYNSSCSKWACVPCRVRSGGGGSGGGGSGGGGSMCQSRYLLFLATLALLNHLSLARVIPVSGPARCLSQSRNLLKTTDDMVKTAREKLKHYSCTAEDIDHEDITRDQTSTLKTCLPLELHKNESCLATRETSSTTRGSCLPPQKTSLMMTLCLGSIYEDLKMYQTEFQAINAALQNHNHQQIILDKGMLVAIDELMQSLNHNGETLRQKPPVGEADPYRVKMKLCILLHAFSTRVVTINRVMGYLSSAGGGGSGGGGSGGGGSGSGATNFSLLKQAGDVEENPGPMRISKPHLRSISIQCYLCLLLNSHFLTEAGIHVFILGCFSAGLPKTEANWVNVISDLKKIEDLIQSMHIDATLYTESDVHPSCKVTAMKCFLLELQVISLESGDASIHDTVENLIILANNSLSSNGNVTESGCKECEELEEKNIKEFLQSFVHIVQMFINTSGGGGSGGGGSGGGGSCGGKVSALKEKVSALKEKVSALKEKVSALKEKVSALKEGGGGSGGGGSGGGGSGSGATNFSLLKQAGDVEENPGPMAPRRARGCRTLGLPALLLLLLLRPPATRGITCPPPMSVEHADIWVKSYSLYSRERYICNSGFKRKAGTSSLTECVLNKATNVAHWTTPSLKCIRDGGGGSGGGGSGGGGSEVSALEKEVSALEKEVSALEKEVSALEKEVSALEK

SEQ ID NO: 571 - protein, 1171 aa, Artificial Sequence
  Synthetic sequence
MCPQKLTISWFAIVLLVSPLMAMWELEKDVYVVEVDWTPDAPGETVNLTCDTPEEDDITWTSDQRHGVIGSGKTLTITVKEFLDAGQYTCHKGGETLSHSHLLLHKKENGIWSTEILKNFKNKTFLKCEAPNYSGRFTCSWLVQRNMDLKFNIKSSSSSPDSRAVTCGMASLSAEKVTLDQRDYEKYSVSCQEDVTCPTAEETLPIELALEARQQNKYENYSTSFFIRDIIKPDPPKNLQMKPLKNSQVEVSWEYPDSWSTPHSYFSLKFFVRIQRKKEKMKETEEGCNQKGAFLVEKTSTEVQCKGGNVCVQAQDRYYNSSCSKWACVPCRVRSGGGGSGGGGSGGGGSMCQSRYLLFLATLALLNHLSLARVIPVSGPARCLSQSRNLLKTTDDMVKTAREKLKHYSCTAEDIDHEDITRDQTSTLKTCLPLELHKNESCLATRETSSTTRGSCLPPQKTSLMMTLCLGSIYEDLKMYQTEFQAINAALQNHNHQQIILDKGMLVAIDELMQSLNHNGETLRQKPPVGEADPYRVKMKLCILLHAFSTRVVTINRVMGYLSSAGGGGSGGGGSGGGGSGSGATNFSLLKQAGDVEENPGPMRISKPHLRSISIQCYLCLLLNSHFLTEAGIHVFILGCFSAGLPKTEANWVNVISDLKKIEDLIQSMHIDATLYTESDVHPSCKVTAMKCFLLELQVISLESGDASIHDTVENLIILANNSLSSNGNVTESGCKECEELEEKNIKEFLQSFVHIVQMFINTSGGGGSGGGGSGGGGSCGGKVSALKEKVSALKEKVSALKEKVSALKEKVSALKEGGGGSGGGGSGGGGSGSGATNFSLLKQAGDVEENPGPMAPRRARGCRTLGLPALLLLLLLRPPATRGITCPPPMSVEHADIWVKSYSLYSRERYICNSGFKRKAGTSSLTECVLNKATNVAHWTTPSLKCIRDPALVHQRPAPPSTVTTAGVTPQPESLSPSGKEPAASSPSSNNTAATTAAIVPGSQLMPSKSPSTGTTEISSHESSHGTPSQTTAKNWELTASASHQPPGVYPQGHSDTTVAISTSTVLLCGLSAVSLLACYLKSRQTPPLASVEMEAMEALPVTWGTSSRDEDLENCSHHLGGGGSGGGGSGGGGSEVSALEKEVSALEKEVSALEKEVSALEKEVSALEK

SEQ ID NO: 572 - DNA, 1230 bp, Herpes Simplex Virus
gtgacgattcccccaatggccgcgcgtcccaggggaggcaggcccaccgcggggcggccccgtccccggggaccaacccggcgcccccaaagaatatcattagcatgcacggcccggcccccgatttgggggcccaacccggtgtcccccaaagaaccccattagcatgcccctcccgccgacgcaacaggggcttggcctgcgtcggtgccccggggcttcccgccttcccgaagaaactcattaccatacccggaaccccaggggaccaatgcgggttcattgagcgacccgcgggccaatgcgcgaggggccgtgtgttccgccaaaaaagcaattagcataacccggaaccccaggggagtggttacgcgcggcgcgggaggcggggaataccggggttgcccattaagggccgcgggaattgccggaagcgggaagggcggccggggccgcccattagttacctgggactgtgcggttgggacggcgcccgtgggcccgggcggccgggggcggcgggggccgcgatggcggcggcggcgggccatggagacagagagcgtgccggggtggtagagtttgacaggcaagcatgtgcgtgcagaggcgagtagtgcttgcctgtctaactcgctagtctcggccgcggggggcccgggctgcccgccgccgccgctttaaagggccgcgcgcgacccccggggggtgtgttttggggggggcccgttttcggggtctggccgctcctccccccgctcctccccccgctcctccccccgctcctccccccgctcctccccccgctcctccccccgctcctccccccgctcctccccccgctcctccccccgctcctccccccgctcctccccccgctcctccccccgctcctccccccgctcctccccccgctcctccccccgctcctccccccgctcctccccccgctcctccccccgctcccgcggccccgccccccacgcccgccgcgcgcgcgcacgccgcccggaccgccgcccgccttttttgcgcgcgcgcgcgcccgcggggggcccgggctgccacaggtgaaaccaacagagcacggcgcactccgcacgtcacacgtcacgtcatccaccacacctgcccaacaacacaactcacagcgacaactcaccgcgcaacaactcctgttcctcatccacacgtcaccgcgcacctcccgctcctccagacgtaccccgg

SEQ ID NO: 573 - DNA, 3185 bp, Herpes Simplex Virus
atgctcgccgtccgttccctgcagcacctctcaaccgtcgtcttgataacggcgtacggcctcgtgctcgtgtggtacaccgtcttcggtgccagtccgctgcaccgatgtatttacgcggtacgccccaccggcaccaacaacgacaccgccctcgtgtggatgaaaatgaaccagaccctattgtttctgggggccccgacgcacccccccaacgggggctggcgcaaccacgcccatatctgctacgccaatcttatcgcgggtagggtcgtgcccttccaggtcccacctgacgccatgaatcgtcggatcatgaacgtccacgaggcagttaactgtctggagaccctatggtacacacgggtgcgtctggtggtcgtagggtggttcctgtatctggcgttcgtcgccctccaccaacgccgatgtatgtttggcgtcgtgagtcccgcccacaagatggtggccccggccacctacctcttgaactacgcaggccgcatcgtatcgagcgtgttcctgcagtacccctacacgaaaattacccgcctgctctgcgagctgtcggtccagcggcaaaacctggttcagttgtttgagacggacccggtcaccttcttgtaccaccgccccgccatcggggtcatcgtaggctgcgagttgatgctacgctttgtggccgtgggtctcatcgtcggcaccgctttcatatcccggggggcatgtgcgatcacataccccctgtttctgaccatcaccacctggtgttttgtctccaccatcggcctgacagagctgtattgtattctgcggcggggcccggcccccaagaacgcagacaaggccgccgccccggggcgatccaaggggctgtcgggcgtctgcgggcgctgctgttccatcatcctctcgggcatcgcagtgcgattgtgttatatcgccgtggtggccggggtggtgctcgtggcgcttcactacgagcaggagatccagaggcgcctgtttgatgtatgacgtcacatccaggccggcggaaaccgtaacggcatatgcaaattggaaactgtcctgtcttggggcccacccacccgacgcgtcatatgcaaatgaaaatcggtcccccgaggccacgtgtagcctggatcccaacgaccccgcccatgggtcccaattggccgtcccgttaccaagaccaacccagccagcatatccacccccgcccgggtccccgcggaagcggaacggggtatgtgatatgctaattaaatacgggaatttccggggactttccgggaatttccggggactttccgggaatttccctacagaggtgcatattaacagagcttttgtcctggagaatgccacgtacttatggtgtctgattggtccttgtctgtgccggaggtggggcgggggccccgcccggggggcggaacgaggaggggtttgggagagccggccccggcaccacgggtataaggacatccaccacccggccggtggtggtgtgcagccgtgttccaaccacggtcacgcttcggtgcctctccccgattcgggcccggtcgctcgctaccggtgcgccaccaccagaggccatatccgacaccccagccccgacggcagccgacagcccggtcatggcgactgacattgatatgctaattgacctcggcctggacctctccgacagcgatctggacgaggacccccccgagccggcggagagccgccgcgacgacctggaatcggacagcagcggggagtgttcctcgtcggacgaggacatggaagacccccacggagaggacggaccggagccgatactcgacgccgctcgcccggcggtccgcccgtctcgtccagaagaccccggcgtacccagcacccagacgcctcgtccgacggagcggcagggccccaacgatcctcaaccagcgccccacagtgtgtggtcgcgcctcggggcccggcgaccgtcttgctcccccgagcagcacgggggcaaggtggcccgcctccaacccccaccgaccaaagcccagcctgcccgcggcggacgccgtgggcgtcgcaggggtcggggtcgcggtggtcccggggctgccgatggtttgtcggacccccgccggcgtgcccccagaaccaatcgcaaccctgggggaccccgccccggggcggggtggacggacggccccggcgccccccatggcgaggcgtggcgcggcagtgagcagcccgacccacccggaggccagcggacacggggcgtgcgccaagcaccccccccgctaatgacgctggcgattgcccccccgcccgcggacccccgcgccccggccccggagcgaaaggcgcccgccgccgacaccatcgacgccaccacgcggttggtcctgcgctccatctccgagcgcgcggcggtcgaccgcatcagcgagagctttggccgcagcgcacaggtcatgcacgacccctttggggggcagccgtttcccgccgcgaatagcccctgggccccggtgctggcgggccaaggagggccctttgacgccgagaccagacgggtctcctgggaaaccttggtcgcccacggcccgagcctctatcgcacttttgccggcaatcctcgggccgcatcgaccgccaaggccatgcgcgactgcgtgctgcgccaagaaaatttcatcgaggcgctggcctccgccgacgagacgctggcgtggtgcaagatgtgcatccaccacaacctgccgctgcgcccccaggaccccattatcgggacggccgcggctgtgctggataacctcgccacgcgcctgcggccctttctccagtgctacctgaaggcgcgaggcctgtgcggcctggacgaactgtgttcgcggcggcgtctggcggacattaaggacattgcatccttcgtgtttgtcattctggccaggctcgccaaccgcgtcgagcgtggcgtcgcggagatcgactacgcgacccttggtgtcggggtcggagagaagatgcatttctacctccccggggcctgcatggcgggcctgatcgaaatcctagacacgcaccgccaggagtgttcgagtcgtgtctgcgagttgacggccagtcacatcgtcgcccccccgtacgtgcacggcaaatatttttattgcaactccctgttttag

SEQ ID NO: 574 - DNA, 3670 bp, Herpes Simplex Virus
atgtcgggcgtcgggggagagggagttccctctgcgcttgcgattctagcctcgtggggctggacgttcgacacgccaaaccacgagtcggggatatcgccagatacgactcccgcagattccattcggggtgccgctgtggcctcacctgaccaacctttacacgggggcccggaacgggaggccacagcgccgtctttctccccaacgcgcgcggatgacggcccgccctgtaccgacgggccctacgtgacgtttgataccctgtttatggtgtcgtcgatcgacgaattagggcgtcgccagctcacggacaccatccgcaaggacctgcggttgtcgctggccaagtttagcattgcgtgcaccaagacctcctcgttttcgggaaacgccccgcgccaccacagacgcggggcgttccagcgcggcacgcgggcgccgcgcagcaacaaaagcctccagatgtttgtgttgtgcaaacgcgcccacgccgctcgagtgcgagagcagcttcgggtcgttattcagtcccgcaagccgcgcaagtattacacgcgatcttcggacgggcggctctgccccgccgtccccgtgttcgtccacgagttcgtctcgtccgagccaatgcgcctccaccgagataacgtcatgctggcctcgggggccgagtaaccgcccccccgcgccaccctcactgcccgtcgcgcgtgtttgatgttaataaataacgcataaatttggctggttgtttgttgtctttaatggaccgcccgcagggggggtggcatttcagtgtcgggtgacgagcgcgatccggccgggagaggctccggtgcccgtcagtgggcagagcgcacatcgcccacagtccccgagaagttggggggaggggtcggcaattgaaccggtgcctagagaaggtggcgcggggtaaactgggaaagtgatgtcgtgtactggctccgcctttttcccgagggtgggggagaaccgtatataagtgcagtagtcgccgtgaacgttctttttcgcaacgggtttgccgccagaacacaggtaagtgccgtgtgtggttcccgcgggcctggcctctttacgggttatggcccttgcgtgccttgaattacttccacgcccctggctgcagtacgtgattcttgatcccgagcttcgggttggaagtgggtgggagagttcgaggccttgcgcttaaggagccccttcgcctcgtgcttgagttgaggcctggcttgggcgctggggccgccgcgtgcgaatctggtggcaccttcgcgcctgtctcgctgctttcgataagtctctagccatttaaaatttttgatgacctgctgcgacgctttttttctggcaagatagtcttgtaaatgcgggccaagatctgcacactggtatttcggtttttggggccgcgggcggcgacggggcccgtgcgtcccagcgcacatgttcggcgaggcggggcctgcgagcgcggccaccgagaatcggacgggggtagtctcaagctggccggcctgctctggtgcctggcctcgcgccgccgtgtatcgccccgccctgggcggcaaggctggcccggtcggcaccagttgcgtgagcggaaagatggccgcttcccggccctgctgcagggagctcaaaatggaggacgcggcgctcgggagagcgggcgggtgagtcacccacacaaaggaaaagggcctttccgtcctcagccgtcgcttcatgtgactccacggagtaccgggcgccgtccaggcacctcgattagttctcgagcttttggagtacgtcgtctttaggttggggggaggggttttatgcgatggagtttccccacactgagtgggtggagactgaagttaggccagcttggcacttgatgtaattctccttggaatttgccctttttgagtttggatcttggttcattctcaagcctcagacagtggttcaaagtttttttcttccatttcaggtgtcgtgagctagcatgtacaggatgcaactcctgtcttgcattgcactaagtcttgcacttgtcacgaattcgatatcgacagcccacccctctcctagcccaagatccgccggccagttcgccatggttagatctcccccatgcccatcatgcccagcacctgagttcctggggggaccatcagtcttcctgttccccccaaaacccaaggacactctcatgatctcccggacccctgaggtcacgtgcgtggtggtggacgtgagccaggaagaccccgaggtccagttcaactggtacgtggatggcgtggaggtgcataatgccaagacaaagccgcgggaggagcagttcaacagcacgtaccgtgtggtcagcgtcctcaccgtcctgcaccaggactggctgaacggcaaggagtacaagtgcaaggtctccaacaaaggcctcccgtcctccatcgagaaaaccatctccaaagccaaagggcagccccgagagccacaggtgtacaccctgcccccatcccaggaggagatgaccaagaaccaggtcagcctgacctgcctggtcaaaggcttctaccccagcgacatcgccgtggagtgggagagcaatgggcagccggagaacaactacaagaccacgcctcccgtgctggactccgacggctccttcttcctctacagcaggctaaccgtggacaagagcaggtggcaggaggggaatgtcttctcatgctccgtgatgcatgaggctctgcacaaccactacacacagaagagcctctccctgtctccgggtaaatgagtggatccaccggatctagataactgatcataatcagccataccacatttgtagaggttttacttgctttaaaaaacctcccacacctccccctgaacctgaaacataaaatgaatgcaattgttgttgttaacttgtttattgcagcttataatggttacaaataaagcaatagcatcacaaatttcacaaataaagcatttttttcactgcattctagttgtggtttgtccaaactcatcaatgtatcttatcctaggaccccaaaagtttgtctgcgtattccagggcggggctcagttgaatctcccgcagcacctctaccagcaggtccgcggtgggctggagaaactcggccgtcccggggcaggcggtcgtcgggggtggaggcgcggcgcccaccccgtgtgccgcgcctggcgtctcctctgggggcgacccgtaaatggttgcagtgatgtaaatggtgtccgcggtccagaccacggtcaaaatgccggccgtggcgctccgggcgctttcgccgcgcgaggagctgacccaggagtcgaacggatacgcgtacatatgggcgtcccacccgcgttcgagcttctggttgctgtcccggcctataaagcggtaggcacaaaattcggcgcgacagtcgataatcaccaacagcccaatgggggtgtgctggataacaacgcctccgcgcggcaggcggtcctggcgctcccggccccgtaccatgatcgcgcgggtgccgtactcaaaaacatgcaccacctgcgcggcgtcgggcagtgcgctggtcagcgaggccctggcgtggcataggctatacgcgatggtcgtctgtggattggacat

SEQ ID NO: 575 - DNA, 6903 bp, Herpes Simplex Virus
ttagaggcgccgggagtggggtcgtcggcgtctgctttttgtggcggcgtcccgtcgcggggtggggtccgacgtggcgatgatgggcggcggcgtggtgaggggcttcggctgcaggcccgcttcatcgtccggcggcagaaccggggtccgtccagacgttccgttggtaggtcccaaatcctgtcgccctacacagcggcgggtgcgcgaatagtcaaagttcacacacccagccttcacaggtgtgtggctggcggcctgcttgcgactgtccagcgcctggcgtatctctttataaagggccaagcgcgtttctgtttcctgggtgttggcaggaaacgcggggtaactcaagtcctccaaaaaacccgccacaaataaaaaggggttaacccaatatgccttctgggcatgcctatcccacaagaccgtgtccaatccgggacagtgataacgcaaaaatataccgtctatcaaagcatagtttatagccgagggggtctcgtaacgccaatcaagatcgtcagacgggagcggcacacaaggcacctttaatatatcccccacctctcgagccacccgactccgaataacatattcggttgaagacaagcccccccgcacacacaaaaccccaacggcaataagcccgacccaacccaaaatccccatagcgcctagggtcggcacccacagaaacctacagtccccaagtgtttgcccagtaacacaaccacgacgtcgtgccacacaagccccgtatccccgttcccgcgcttttcgttggtttatatacacattgattattgactagttattaatagtaatcaattacggggtcattagttcatagcccatatatggagttccgcgttacataacttacggtaaatggcccgcctggctgaccgcccaacgacccccgcccattgacgtcaataatgacgtatgttcccatagtaacgccaatagggactttccattgacgtcaatgggtggagtatttacggtaaactgcccacttggcagtacatcaagtgtatcatatgccaagtacgccccctattgacgtcaatgacggtaaatggcccgcctggcattatgcccagtacatgaccttatgggactttcctacttggcagtacatctacgtattagtcatcgctattaccatggtgatgcggttttggcagtacatcaatgggcgtggatagcggtttgactcacggggatttccaagtctccaccccattgacgtcaatgggagtttgttttggcaccaaaatcaacgggactttccaaaatgtcgtaacaactccgccccattgacgcaaatgggcggtaggcgtgtacggtgggaggtctatataagcagagctctctggctaactagagaacccactgcttactggcttatcgaaattaatacgactcactatagggagacccaagctggctagcgtttaaacttaagcttggtaccgagctcggatccactagtccagtgtggtggaattcgccaccatgtgccatcagcagctggtcatctcatggttctccctggtgtttctggcctcacctctggtcgcaatctgggaactgaaaaaggatgtgtacgtggtggagctggactggtatcccgatgcccctggcgagatggtggtgctgacctgcgacacacccgaggaggatggcatcacctggacactggatcagagctccgaggtgctgggaagcggcaagaccctgacaatccaggtgaaggagttcggcgacgccggccagtacacctgtcacaagggaggagaggtgctgagccactccctgctgctgctgcacaagaaggaggatggcatctggtccacagacatcctgaaggatcagaaggagccaaagaacaagaccttcctgcggtgcgaggccaagaattatagcggccggttcacctgttggtggctgaccacaatctccaccgatctgacattttctgtgaagtctagcaggggatcctctgacccacagggagtgacatgcggagcagccaccctgagcgccgagagggtgcgcggcgataacaaggagtacgagtattccgtggagtgccaggaggactctgcctgtccagcagcagaggagtccctgcctatcgaagtgatggtggatgccgtgcacaagctgaagtacgagaattataccagctccttctttatccgggacatcatcaagcccgatccccctaagaacctgcagctgaagcctctgaagaatagcagacaggtggaggtgtcctgggagtaccctgacacctggagcacaccacactcctatttctctctgaccttttgcgtgcaggtgcagggcaagtccaagcgggagaagaaggacagagtgttcaccgataagacatctgccaccgtgatctgtagaaagaacgcctctatcagcgtgagggcccaggaccgctactattctagctcctggtccgagtgggcctctgtgccttgcagcggcggaggaggaggaggatctatgtgcccagcaaggagcctgctgctggtggccacactggtgctgctggatcacctgtccctggcaaggaatctgccagtggcaacccctgacccaggcatgttcccctgcctgcaccacagccagaacctgctgagggccgtgtccaatatgctgcagaaggcccgccagacactggagttttacccttgtaccagcgaggagatcgaccacgaggacatcacaaaggataagacctccacagtggaggcctgcctgccactggagctgaccaagaacgagtcctgtctgaacagccgggagacaagcttcatcaccaacggctcctgcctggcctctagaaagacaagctttatgatggccctgtgcctgtctagcatctacgaggacctgaagatgtatcaggtggagttcaagaccatgaacgccaagctgctgatggaccccaagaggcagatctttctggatcagaatatgctggccgtgatcgacgagctgatgcaggccctgaacttcaatagcgagacagtgcctcagaagtcctctctggaggagccagatttctacaagaccaagatcaagctgtgcatcctgctgcacgcctttcggatcagagccgtgacaatcgaccgcgtgatgtcctatctgaacgcctctggaggaggaggaagcggaggaggaggatccggcggcggcggctccggctctggcgccaccaacttctccctgctgaagcaggcaggcgacgtggaggagaatccaggacctatgcggatctctaagcctcacctgagaagcatctccatccagtgctacctgtgcctgctgctgaacagccactttctgacagaggccggcatccacgtgttcatcctgggctgttttagcgccggcctgccaaagaccgaggcaaactgggtgaatgtgatctctgacctgaagaagatcgaggatctgatccagagcatgcacatcgatgccacactgtataccgagtctgacgtgcaccctagctgcaaggtgaccgccatgaagtgtttcctgctggagctgcaggtcatcagcctggagtccggcgacgcaagcatccacgatacagtggagaacctgatcatcctggccaacaatagcctgagctccaacggcaatgtgaccgagtccggctgcaaggagtgtgaggagctggaggagaagaacatcaaggagttcctgcagagctttgtgcacatcgtgcagatgttcatcaatacatccggaggaggaggatcaggcggaggaggaagcggcggcggcggctctggcagcggcgccaccaacttttccctgctgaagcaggccggcgatgtggaagaaaatccaggaccaatggcaccaaggagagcaaggggatgcagaaccctgggcctgcctgccctgttattactgctgctgctgaggccaccagcaacaaggggaatcacctgtcctccacccatgagcgtggagcacgccgacatctgggtgaagtcctactctctgtattctagggagcggtacatctgcaacagcggctttaagaggaaggccggcacatctagcctgaccgagtgcgtgctgaacaaggccaccaatgtggcccactggaccacaccttccctgaagtgcatcagggatccagccctggtgcaccagcgccccgcacctccaagcacagtgaccacagcaggagtgacccctcagccagagagcctgtccccttctggcaaggagccagcagcatcctctccaagctccaacaatacagcagcaaccacagcagcaatcgtgccaggctcccagctgatgccaagcaagtccccctctaccggcaccacagagatctctagccacgagtcctctcacggcacaccaagccagaccacagccaagaattgggagctgaccgcaagcgcctcccaccagccacctggcgtgtacccacagggacactccgacaccacagtggccatctctaccagcacagtgctgctgtgcggcctgtctgccgtgagcctgctggcctgttatctgaagtccaggcagaccccaccactggcatctgtggagatggaggccatggaggccctgcccgtcacatgggggactagtagtagagacgaggatctggaaaactgtagtcaccatctgtaagatatccatcacactggcggccgctcgagcatgcatctagagggccctattctatagtgtcacctaaatgctagagctcgctgatcagcctcgactgtgccttctagttgccagccatctgttgtttgcccctcccccgtgccttccttgaccctggaaggtgccactcccactgtcctttcctaataaaatgaggaaattgcatcgcattgtctgagtaggtgtcattctattctggggggtggggtggggcaggacagcaagggggaggattgggaagacaatagcaggcatgctggggatgcggtgggctctatggggatccactagttctagagcggccgccgcacataaaggcccggcgcgaccgacgcccgcagacggcgccggccacgaacgacgggagcggctgcggagcacgcggaccgggagcgggactcgcagagggccgtcggagcggacggcgtcggcatcgcgacgccccggctcgggatcgggatcgcatcggaaagggacacgcggaaagacccacccaccccacccacgaaacacaggggacgcaccccgggggcctccgacgacagaaacccaccggtccgcctttgtgcacgggtaagcaccttgggtgggcggaggaggggggacgcgggggcggaggagggggctcacccgcgttcgtgccttcccgcaggaggaacgtcctcgtcgaggcgaccggcggcgaccgttgcgtggaccgcttcctgctcgtcggggcgaccggcggcgaccgttgcgtggaccgcttcctgctcgtcgggcgggggagcatgtcgtgggccctggaaatggcggacaccttcctggacaacatgcgggttgggcccaggacgtacgccgacgtacgcgatgagatcaataaaagggggcgtgaggaccgggaggcggccaaaaccgccgtgcacgacccggagcgtcctctgctgcgctctcccgggctgctgcccaaaatcgcccccaacgcatccttgggtgtggcacatcgaagaaccggcgggaccgtgaccgacagtccccgtaatccggtaacccgttgagtcccgggtacgaccatcgcccaagtttctgggcggagggtggttccccccgtggctctcgagatgagccagacccaacccccggccccagttgggccgggcgacccagatgtttacttaaaaggcgtgccgtccgccggcatgcaccccagaggtgttcacgcacctcgaggacacccgcgcatgatctccggacccccgcaacggggtgataatgatcaagcggcggggcaatgtggagattcgggtctactacgagtcggtgcggacactacgatctcgaagccatctgaagccgtccgaccgccaacaatccccaggacaccgcgtgttccccgggagccccgggttccgcgaccaccccgagaacctagggaacccagagtaccgcgagctcccagagaccccagggtaccgcgtgaccccagggatccacgacaaccccgggagccccggcctccccgggagccccggaccccacgcaccccccgcgaaccacgtacggctcgcgggtctgtatagcccgggcaagtatgcccccctggcgagcccagaccccttctccccacaagatggagcgtacgctcgggcccgcgtagggctccacaccgcggttcgcgtcccgcccaccggaagcccaacccacacgcacttgcggcatgacccgggcgatgagccaacctcggatgactcagggctctaccctctggacgcccgggcgcttgcgcacctggtgatgttgcccgcggaccaccgggccttctttcgaaccgtggtcgaggtgtctcgcatgtgcgctgcaaacgtgcgcgatcccccgcccccggctacaggggccatgttgggccgccacgcgcggctggtccacacccagtggctccgggccaaccaagagacgtcgcccctgtggccctggcggacggcggccattaactttatcaccaccatggccccccgcgtccaaacccaccgacacatgcacgacctgttgatggcctgtgctttctggtgctgtctgacacacgcatcgacgtgttcgtacgcggggctgtactcgacccactgcctgcatctgtttggtgcgtttgggtgtggggacccggccctaaccccacccctgtgctag